European Patent Application EP 4 636 089 A1, published October 22, 2025. Title: Nucleic acid construct capagle of selectively detecting or killing mispatch repair-deficient cells and use of the same. Applicant: 公立大学法人横浜市立大学. Application JP. The sequence listing filed with the application follows.

SEQUENCE LISTING (234 sequences)

SEQ ID NO: 1 - DNA, 23 bp, synthetic construct
  source 1..23: mol_type = other DNA; note = primer Nluc-Fw
taatacgactcactataggctag

SEQ ID NO: 2 - DNA, 43 bp, synthetic construct
  source 1..43: mol_type = other DNA; note = primer Sce-5'Nluc-Rv
attaccctgttatccctatcactggcccatttggtcgccgctc

SEQ ID NO: 3 - DNA, 45 bp, synthetic construct
  source 1..45: mol_type = other DNA; note = primer Sce-3'Nluc-Fw
tgatagggataacagggtaatgtgtaccctgtggatgatcatcac

SEQ ID NO: 4 - DNA, 23 bp, synthetic construct
  source 1..23: mol_type = other DNA; note = primer Nluc-Rv
ccgccccgactctagagtcgcgg

SEQ ID NO: 5 - DNA, 44 bp, synthetic construct
  source 1..44: mol_type = other DNA; note = primer iNluc-Fw
aaatcgataaggatcgctagcatgaagatttcgttggggactgg

SEQ ID NO: 6 - DNA, 44 bp, synthetic construct
  source 1..44: mol_type = other DNA; note = primer iNluc-Rv
caccatacgcggatccttatcagttgatggttactcggaacagc

SEQ ID NO: 7 - DNA, 516 bp, synthetic construct
  source 1..516: mol_type = other DNA; note = NanoLuc (Nluc) gene encoding modified luciferase
  CDS 1..516: protein_id = 8; translation = MVFTLEDFVGDWRQTAGYNLDQVLEQGGVSSLFQNLGVSVTPIQRIVLSGENGLKIDIHVIIPYEGLSGDQMGQIEKIFKVVYPVDDHHFKVILHYGTLVIDGVTPNMIDYFGRPYEGIAVFDGKKITVTGTLWNGNKIIDERLINPDGSLLFRVTINGVTGWRLCERILA
atggtcttcacactcgaagatttcgttggggactggcgacagacagccggctacaacctggaccaagtccttgaacagggaggtgtgtccagtttgtttcagaatctcggggtgtccgtaactccgatccaaaggattgtcctgagcggtgaaaatgggctgaagatcgacatccatgtcatcatcccgtatgaaggtctgagcggcgaccaaatgggccagatcgaaaaaatttttaaggtggtgtaccctgtggatgatcatcactttaaggtgatcctgcactatggcacactggtaatcgacggggttacgccgaacatgatcgactatttcggacggccgtatgaaggcatcgccgtgttcgacggcaaaaagatcactgtaacagggaccctgtggaacggcaacaaaattatcgacgagcgcctgatcaaccccgacggctccctgctgttccgagtaaccatcaacggagtgaccggctggcggctgtgcgaacgcattctggcgtaa

SEQ ID NO: 8 - protein, 171 aa, synthetic construct
MVFTLEDFVGDWRQTAGYNLDQVLEQGGVSSLFQNLGVSVTPIQRIVLSGENGLKIDIHVIIPYEGLSGDQMGQIEKIFKVVYPVDDHHFKVILHYGTLVIDGVTPNMIDYFGRPYEGIAVFDGKKITVTGTLWNGNKIIDERLINPDGSLLFRVTINGVTGWRLCERILA

SEQ ID NO: 9 - DNA, 516 bp, synthetic construct
  source 1..516: mol_type = other DNA; note = SceNluc gene
  CDS 1..225: protein_id = 10; translation = MVFTLEDFVGDWRQTAGYNLDQVLEQGGVSSLFQNLGVSVTPIQRIVLSGENGLKIDIHVIIPYEGLSGDQMGQ
  CDS 235..516: protein_id = 11; translation = QGNVYPVDDHHFKVILHYGTLVIDGVTPNMIDYFGRPYEGIAVFDGKKITVTGTLWNGNKIIDERLINPDGSLLFRVTINGVTGWRLCERILA
atggtcttcacactcgaagatttcgttggggactggcgacagacagccggctacaacctggaccaagtccttgaacagggaggtgtgtccagtttgtttcagaatctcggggtgtccgtaactccgatccaaaggattgtcctgagcggtgaaaatgggctgaagatcgacatccatgtcatcatcccgtatgaaggtctgagcggcgaccaaatgggccagtgatagggataacagggtaatgtgtaccctgtggatgatcatcactttaaggtgatcctgcactatggcacactggtaatcgacggggttacgccgaacatgatcgactatttcggacggccgtatgaaggcatcgccgtgttcgacggcaaaaagatcactgtaacagggaccctgtggaacggcaacaaaattatcgacgagcgcctgatcaaccccgacggctccctgctgttccgagtaaccatcaacggagtgaccggctggcggctgtgcgaacgcattctggcgtaa

SEQ ID NO: 10 - protein, 74 aa, synthetic construct
MVFTLEDFVGDWRQTAGYNLDQVLEQGGVSSLFQNLGVSVTPIQRIVLSGENGLKIDIHVIIPYEGLSGDQMGQ

SEQ ID NO: 11 - protein, 93 aa, synthetic construct
QGNVYPVDDHHFKVILHYGTLVIDGVTPNMIDYFGRPYEGIAVFDGKKITVTGTLWNGNKIIDERLINPDGSLLFRVTINGVTGWRLCERILA

SEQ ID NO: 12 - DNA, 462 bp, synthetic construct
  source 1..462: mol_type = other DNA; note = iNluc gene (homology 100%)
  CDS 1..462: protein_id = 13; translation = EDFVGDWRQTAGYNLDQVLEQGGVSSLFQNLGVSVTPIQRIVLSGENGLKIDIHVIIPYEGLSGDQMGQIEKIFKVVYPVDDHHFKVILHYGTLVIDGVTPNMIDYFGRPYEGIAVFDGKKITVTGTLWNGNKIIDERLINPDGSLLFRVTIN
gaagatttcgttggggactggcgacagacagccggctacaacctggaccaagtccttgaacagggaggtgtgtccagtttgtttcagaatctcggggtgtccgtaactccgatccaaaggattgtcctgagcggtgaaaatgggctgaagatcgacatccatgtcatcatcccgtatgaaggtctgagcggcgaccaaatgggccagatcgaaaaaatttttaaggtggtgtaccctgtggatgatcatcactttaaggtgatcctgcactatggcacactggtaatcgacggggttacgccgaacatgatcgactatttcggacggccgtatgaaggcatcgccgtgttcgacggcaaaaagatcactgtaacagggaccctgtggaacggcaacaaaattatcgacgagcgcctgatcaaccccgacggctccctgctgttccgagtaaccatcaactga

SEQ ID NO: 13 - protein, 153 aa, synthetic construct
EDFVGDWRQTAGYNLDQVLEQGGVSSLFQNLGVSVTPIQRIVLSGENGLKIDIHVIIPYEGLSGDQMGQIEKIFKVVYPVDDHHFKVILHYGTLVIDGVTPNMIDYFGRPYEGIAVFDGKKITVTGTLWNGNKIIDERLINPDGSLLFRVTIN

SEQ ID NO: 14 - DNA, 459 bp, synthetic construct
  source 1..459: mol_type = other DNA; note = iNluc gene (homology 95%)
gaagatttcgttggcgactggcgacagacagctggctacaacctggaccaggtccttgaacagggaggcgtgtccagtttgtttcaaaatctcggggtgtccgtgactccgatccaaaggatcgtcctgagcggtgaaaacgggctgaagatcgacattcatgtcatcatcccgtacgaaggtctgagcggcgatcaaatgggccagatcgaaaaaatttttaaggtggtgtaccctgtggatgaccatcactttaaggtgattctgcactatggcacactcgtaatcgacggggttaccccgaacatgatcgactacttcggacggccgtatgagggcatcgccgtgttcgatggcaaaaagatcactgtgacagggaccctgtggaatggcaacaaaattatcgatgagcgcctgatcaaccctgacggctccctgctgtttcgagtaaccatcaac

SEQ ID NO: 15 - DNA, 459 bp, synthetic construct
  source 1..459: mol_type = other DNA; note = iNluc gene (homology 90%)
gaagatttcgttggcgactggcggcagacagctggctacaatctggaccaggtccttgagcagggaggcgtgtccagcttgtttcaaaatctcggcgtgtccgtgactccgattcaaaggatcgtcctgagtggtgaaaacgggctgaaaatcgacattcatgtcattatcccgtacgaaggtctcagcggcgatcaaatgggccagatcgaaaaaatttttaaggtggtgtaccctgtggacgatcatcattttaaggtcatcctgcattatggcaccctggtaattgacggggtgacgccgaatatgatcgattatttcggccggccgtacgaaggcattgccgtgtttgacggcaagaagatcaccgtaacaggcaccctgtggaacggcaataaaattattgacgagcggctgatcaatcccgacgggtccctgctcttccgagtgaccatcaac

SEQ ID NO: 16 - DNA, 459 bp, synthetic construct
  source 1..459: mol_type = other DNA; note = iNluc gene (homology 80%)
gaggacttcgtgggcgactggcggcagaccgctggctataatctggatcaggtcctggagcagggcggcgtgtctagcttgttccaaaatctgggcgtgtctgtgactcccattcaaagaatcgtcctcagtggtgagaacgggctcaaaatcgatattcatgtgattatcccctacgaaggcctcagcggggatcaaatggggcagatcgaaaaaatttttaaggtggtctatcctgtcgacgatcaccattttaaagtcatcctccattatggaaccctggtgattgacggcgtgacgcccaatatgattgattattttggccggccctacgaagggattgccgtctttgacgggaagaagattaccgtaaccggcaccctctggaacgggaataaaatcattgacgaacggctgattaatcccgatgggtccctcctcttccgggtgaccattaac

SEQ ID NO: 17 - DNA, 459 bp, synthetic construct
  source 1..459: mol_type = other DNA; note = iNluc gene (homology 70%)
gaggactttgtgggcgattggcggcaaaccgctgggtataatctcgatcaggtgctggagcaaggcggcgtctctagcttattccaaaacctgggcgtctctgtgacccccattcagagaatcgtgctcagtggcgagaacggcctcaaaattgatattcacgtgattattccctacgagggcctcagtggggatcagatggggcagatcgaaaaaatttttaaggtggtctatcccgtcgacgaccaccatttcaaagtcattctccattacggaaccctcgtgattgatggcgtgacccccaatatgattgattactttggccgcccctacgaggggattgctgtctttgatgggaagaaaattaccgtgaccggcacactctggaatgggaataagatcattgatgaacggctcattaatcctgatgggtctctcctctttcgggtgacaattaac

SEQ ID NO: 18 - DNA, 459 bp, synthetic construct
  source 1..459: mol_type = other DNA; note = iNluc gene (homology 99%)
gaagatttcgttggggactggcgacagacagccggctacaacctggaccaagtccttgaacagggaggcgtgtccagtttgtttcagaatctcggggtgtccgtaactccgatccaaaggattgtcctgagcggtgagaatgggctgaagatcgacatccatgtcatcatcccgtatgaaggtctgagcggcgaccaaatgggccagatcgaaaaaatttttaaggtggtgtaccctgtggatgatcatcactttaaggtgatcctgcactatggcacactggtaatcgacggggttacgccgaatatgatcgactatttcggacggccgtatgaaggcatcgccgtgttcgacggcaaaaagatcactgtaacagggacactgtggaacggcaacaaaattatcgacgagcgcctgatcaaccccgacggctccctgctgttccgagtaaccatcaac

SEQ ID NO: 19 - DNA, 459 bp, synthetic construct
  source 1..459: mol_type = other DNA; note = iNluc gene (homology 98%)
gaagatttcgttggggactggcgacagacagccggctacaatctggaccaagtccttgaacagggaggtgtgtccagtttgttccagaatctcggggtgtccgtaactccgatccaaaggatcgtcctgagcggtgaaaatgggctgaagatcgacatccatgtgatcatcccgtatgaaggtctgagcggcgaccaaatgggccagatcgaaaaaatttttaaggtggtgtaccctgtggatgatcatcactttaaggtgatcctgcactatgggacactggtaatcgacggggttacgccgaacatgatcgactattttggacggccgtatgaaggcatcgccgtgttcgacggcaaaaagattactgtaacagggaccctgtggaacggcaacaaaattatcgacgaacgcctgatcaaccccgacggctccctgctgttccgagtaaccatcaac

SEQ ID NO: 20 - DNA, 459 bp, synthetic construct
  source 1..459: mol_type = other DNA; note = iNluc gene (homology 97%)
gaagatttcgttggggactggcgacagaccgccggctacaacctggaccaagtccttgagcagggaggtgtgtccagtttgtttcagaacctcggggtgtccgtaactccgatccagaggattgtcctgagcggtgaaaatgggctcaagatcgacatccatgtcatcatcccgtacgaaggtctgagcggcgaccaaatgggccagatcgaaaaaatttttaaggtggtgtaccctgtggatgatcatcactttaaagtgatcctgcactatggcacactggtgatcgacggggttacgccgaacatgatcgattatttcggacggccgtatgaaggcattgccgtgttcgacggcaaaaagatcactgtgacagggaccctgtggaacggcaacaagattatcgacgagcgcctgatcaaccccgatggctccctgctgttccgagtaaccatcaac

SEQ ID NO: 21 - DNA, 459 bp, synthetic construct
  source 1..459: mol_type = other DNA; note = iNluc gene (homology 96%)
gaagatttcgttggggactggcggcagacagccggctacaacctggatcaagtccttgaacagggaggcgtgtccagtttgtttcagaatctgggggtgtccgtaactccgattcaaaggattgtcctgagcggtgagaatgggctgaagatcgacattcatgtcatcatcccgtatgaaggcctgagcggcgaccaaatgggccagatcgaaaaaatttttaaggtggtgtaccctgtggatgatcatcattttaaggtgatcctgcactacggcacactggtaatcgacggggtgacgccgaacatgatcgactattttggacggccgtatgaaggcattgccgtgttcgacggcaaaaagataactgtaacagggaccctgtggaatggcaacaaaattatcgacgaacgcctgatcaaccccgacggctctctgctgttccgagtaaccatcaac

SEQ ID NO: 22 - DNA, 459 bp, synthetic construct
  source 1..459: mol_type = other DNA; note = iNluc gene (homology 94%)
gaagatttcgttggggattggcgacagacagctggctacaacctggatcaagtccttgaacaaggaggtgtgtccagtttatttcagaatctcggcgtgtccgtaactcccatccaaaggattgtgctgagcggtgaaaatggcctgaagatcgacattcatgtcatcatcccctatgaaggtctgagtggcgaccaaatgggccagatcgaaaaaatttttaaggtggtgtaccctgtggatgaccatcactttaaggtcatcctgcactatgggacactggtaatcgatggggttacgccgaatatgatcgactattttggacggccgtatgagggcatcgccgtgtttgacggcaaaaagataactgtaacagggacactgtggaacggcaataaaattatcgacgaacgcctgatcaaccctgacggctccctgctcttccgagtaaccatcaac

SEQ ID NO: 23 - DNA, 33 bp, synthetic construct
  source 1..33: mol_type = other DNA; note = primer NlucP-Rv
gccgtgagaattcgccagaatgcgttcgcacag

SEQ ID NO: 24 - DNA, 30 bp, synthetic construct
  source 1..30: mol_type = other DNA; note = primer hPEST-Fw
ttctggcgaattctcacggctttccgcctg

SEQ ID NO: 25 - DNA, 42 bp, synthetic construct
  source 1..42: mol_type = other DNA; note = primer hPEST-Rv
cggccgccccgactctagattagacgttgatgcgagctgaag

SEQ ID NO: 26 - DNA, 120 bp, synthetic construct
  source 1..120: mol_type = other DNA; note = 120 bp hPEST fragment
  CDS 1..120: protein_id = 27; translation = SHGFPPEVEEQAAGTLPMSCAQESGMDRHPAACASARINV
tctcacggctttccgcctgaggttgaagagcaagccgccggtacattgcctatgtcctgcgcacaagaaagcggtatggaccggcacccagccgcttgtgcttcagctcgcatcaacgtc

SEQ ID NO: 27 - protein, 40 aa, synthetic construct
SHGFPPEVEEQAAGTLPMSCAQESGMDRHPAACASARINV

SEQ ID NO: 28 - DNA, 639 bp, synthetic construct
  source 1..639: mol_type = other DNA
  CDS 1..639: protein_id = 29; translation = MVFTLEDFVGDWRQTAGYNLDQVLEQGGVSSLFQNLGVSVTPIQRIVLSGENGLKIDIHVIIPYEGLSGDQMGQIEKIFKVVYPVDDHHFKVILHYGTLVIDGVTPNMIDYFGRPYEGIAVFDGKKITVTGTLWNGNKIIDERLINPDGSLLFRVTINGVTGWRLCERILANSHGFPPEVEEQAAGTLPMSCAQESGMDRHPAACASARINV
atggtcttcacactcgaagatttcgttggggactggcgacagacagccggctacaacctggaccaagtccttgaacagggaggtgtgtccagtttgtttcagaatctcggggtgtccgtaactccgatccaaaggattgtcctgagcggtgaaaatgggctgaagatcgacatccatgtcatcatcccgtatgaaggtctgagcggcgaccaaatgggccagatcgaaaaaatttttaaggtggtgtaccctgtggatgatcatcactttaaggtgatcctgcactatggcacactggtaatcgacggggttacgccgaacatgatcgactatttcggacggccgtatgaaggcatcgccgtgttcgacggcaaaaagatcactgtaacagggaccctgtggaacggcaacaaaattatcgacgagcgcctgatcaaccccgacggctccctgctgttccgagtaaccatcaacggagtgaccggctggcggctgtgcgaacgcattctggcgaattctcacggctttccgcctgaggttgaagagcaagccgccggtacattgcctatgtcctgcgcacaagaaagcggtatggaccggcacccagccgcttgtgcttcagctcgcatcaacgtctaa

SEQ ID NO: 29 - protein, 212 aa, synthetic construct
MVFTLEDFVGDWRQTAGYNLDQVLEQGGVSSLFQNLGVSVTPIQRIVLSGENGLKIDIHVIIPYEGLSGDQMGQIEKIFKVVYPVDDHHFKVILHYGTLVIDGVTPNMIDYFGRPYEGIAVFDGKKITVTGTLWNGNKIIDERLINPDGSLLFRVTINGVTGWRLCERILANSHGFPPEVEEQAAGTLPMSCAQESGMDRHPAACASARINV

SEQ ID NO: 30 - DNA, 639 bp, synthetic construct
  source 1..639: mol_type = other DNA
  CDS 1..225: protein_id = 31; translation = MVFTLEDFVGDWRQTAGYNLDQVLEQGGVSSLFQNLGVSVTPIQRIVLSGENGLKIDIHVIIPYEGLSGDQMGQ
  CDS 235..639: protein_id = 32; translation = QGNVYPVDDHHFKVILHYGTLVIDGVTPNMIDYFGRPYEGIAVFDGKKITVTGTLWNGNKIIDERLINPDGSLLFRVTINGVTGWRLCERILANSHGFPPEVEEQAAGTLPMSCAQESGMDRHPAACASARINV
atggtcttcacactcgaagatttcgttggggactggcgacagacagccggctacaacctggaccaagtccttgaacagggaggtgtgtccagtttgtttcagaatctcggggtgtccgtaactccgatccaaaggattgtcctgagcggtgaaaatgggctgaagatcgacatccatgtcatcatcccgtatgaaggtctgagcggcgaccaaatgggccagtgatagggataacagggtaatgtgtaccctgtggatgatcatcactttaaggtgatcctgcactatggcacactggtaatcgacggggttacgccgaacatgatcgactatttcggacggccgtatgaaggcatcgccgtgttcgacggcaaaaagatcactgtaacagggaccctgtggaacggcaacaaaattatcgacgagcgcctgatcaaccccgacggctccctgctgttccgagtaaccatcaacggagtgaccggctggcggctgtgcgaacgcattctggcgaattctcacggctttccgcctgaggttgaagagcaagccgccggtacattgcctatgtcctgcgcacaagaaagcggtatggaccggcacccagccgcttgtgcttcagctcgcatcaacgtctaa

SEQ ID NO: 31 - protein, 74 aa, synthetic construct; identical to SEQ ID NO: 10

SEQ ID NO: 32 - protein, 134 aa, synthetic construct
QGNVYPVDDHHFKVILHYGTLVIDGVTPNMIDYFGRPYEGIAVFDGKKITVTGTLWNGNKIIDERLINPDGSLLFRVTINGVTGWRLCERILANSHGFPPEVEEQAAGTLPMSCAQESGMDRHPAACASARINV

SEQ ID NO: 33 - DNA, 48 bp, synthetic construct
  source 1..48: mol_type = other DNA; note = primer 5'SceNluc3-Rv
cattaccctgttatccctacgcgtcaaccgctcaggacaatcctttgg

SEQ ID NO: 34 - DNA, 47 bp, synthetic construct
  source 1..47: mol_type = other DNA; note = primer 3'SceNluc3-Fw
gtagggataacagggtaatgcatatatcgacgagcgcctgatcaacc

SEQ ID NO: 35 - DNA, 22 bp, synthetic construct
  source 1..22: mol_type = other DNA; note = primer iNluc3-1-100-Fw
agaatctcggggtgtccgtaac

SEQ ID NO: 36 - DNA, 24 bp, synthetic construct
  source 1..24: mol_type = other DNA; note = primer iNluc3-1-100-Rv
ttcggcgtaaccccgtcgattacc

SEQ ID NO: 37 - DNA, 23 bp, synthetic construct
  source 1..23: mol_type = other DNA; note = primer iNluc3-2-100-Fw
aaggtgatcctgcactatggcac

SEQ ID NO: 38 - DNA, 25 bp, synthetic construct
  source 1..25: mol_type = other DNA; note = primer iNluc3-2-100-Rv
ttactcggaacagcagggagccgtc

SEQ ID NO: 39 - DNA, 49 bp, synthetic construct
  source 1..49: mol_type = other DNA; note = primer iNluc3-1-90-Fw
agaatctgggggtgtctgtaactcccatccaaagaattgtcctcagcgg

SEQ ID NO: 40 - DNA, 27 bp, synthetic construct
  source 1..27: mol_type = other DNA; note = primer iNluc3-1-90-Rv
ttcggggtaaccccatcgattacgagt

SEQ ID NO: 41 - DNA, 50 bp, synthetic construct
  source 1..50: mol_type = other DNA; note = primer iNluc3-1-80-Fw
agaacctcggcgtctctgtaaccccgattcaaagaatcgtgctgagtggt

SEQ ID NO: 42 - DNA, 26 bp, synthetic construct
  source 1..26: mol_type = other DNA; note = primer iNluc3-1-80-Rv
ttgggcgtcacgccatcgatcaccag

SEQ ID NO: 43 - DNA, 25 bp, synthetic construct
  source 1..25: mol_type = other DNA; note = primer iNluc3-2-90-Fw
aaggtgattctgcactacggcacac

SEQ ID NO: 44 - DNA, 28 bp, synthetic construct
  source 1..28: mol_type = other DNA; note = primer iNluc3-2-90-Rv
aaggtcatcctccattacggcaccctgg

SEQ ID NO: 45 - DNA, 48 bp, synthetic construct
  source 1..48: mol_type = other DNA; note = primer iNluc3-2-80-Fw
ttactcgaaacagcagagagccgtcagggttgatgaggcgctcatcga

SEQ ID NO: 46 - DNA, 50 bp, synthetic construct
  source 1..50: mol_type = other DNA; note = primer iNluc3-2-80-Rv
ttacccggaagaggagagagccatcgggattgatgagccgttcgtcaata

SEQ ID NO: 47 - DNA, 280 bp, synthetic construct
  source 1..280: mol_type = other DNA; note = SceNluc3 gene
atggtcttcacactcgaagatttcgttggggactggcgacagacagccggctacaacctggaccaagtccttgaacagggaggtgtgtccagtttgtttcagaatctcggggtgtccgtaactccgatccaaaggattgtcctgagcggttgacgcgtagggataacagggtaatgcatatatcgacgagcgcctgatcaaccccgacggctccctgctgttccgagtaaccatcaacggagtgaccggctggcggctgtgcgaacgcattctggcgtaa

SEQ ID NO: 48 - DNA, 220 bp, synthetic construct
  source 1..220: mol_type = other DNA; note = iNluc3-1-100 fragment
agaatctcggggtgtccgtaactccgatccaaaggattgtcctgagcggtgaaaatgggctgaagatcgacatccatgtcatcatcccgtatgaaggtctgagcggcgaccaaatgggccagatcgaaaaaatttttaaggtggtgtaccctgtggatgatcatcactttaaggtgatcctgcactatggcacactggtaatcgacggggttacgccgaa

SEQ ID NO: 49 - DNA, 196 bp, synthetic construct
  source 1..196: mol_type = other DNA; note = iNluc3-2-100 fragment
aaggtgatcctgcactatggcacactggtaatcgacggggttacgccgaacatgatcgactatttcggacggccgtatgaaggcatcgccgtgttcgacggcaaaaagatcactgtaacagggaccctgtggaacggcaacaaaattatcgacgagcgcctgatcaaccccgacggctccctgctgttccgagtaa

SEQ ID NO: 50 - DNA, 220 bp, synthetic construct
  source 1..220: mol_type = other DNA; note = iNluc3-1-90 fragment
agaatctgggggtgtctgtaactcccatccaaagaattgtcctcagcggtgaaaatgggctgaagatcgacatccatgtcatcatcccgtatgaaggtctgagcggcgaccaaatgggccagatcgaaaaaatttttaaggtggtgtaccctgtggatgatcatcactttaaggtgatcctgcactatggcacactcgtaatcgatggggttaccccgaa

SEQ ID NO: 51 - DNA, 219 bp, synthetic construct
  source 1..219: mol_type = other DNA; note = iNluc3-1-80 fragment
agaacctcggcgtctctgtaaccccgattcaaagaatcgtgctgagtggtgaaaatgggctgaagatcgacatccatgtcatcatcccgtatgaaggtctgagcggcgaccaaatgggccagatcgaaaaaatttttaaggtggtgtaccctgtggatgatcatcactttaaggtgatcctgcactatggcacctggtgatcgatggcgtgacgcccaa

SEQ ID NO: 52 - DNA, 196 bp, synthetic construct
  source 1..196: mol_type = other DNA; note = iNluc3-2-90 fragment
aaggtgattctgcactacggcacactggtaatcgacggggttacgccgaacatgatcgactatttcggacggccgtatgaaggcatcgccgtgttcgacggcaaaaagatcactgtaacagggaccctgtggaacggcaacaaaattatcgatgagcgcctcatcaaccctgacggctctctgctgtttcgagtaa

SEQ ID NO: 53 - DNA, 196 bp, synthetic construct
  source 1..196: mol_type = other DNA; note = iNluc3-2-80 fragment
aaggtcatcctccattacggcaccctggtaatcgacggggttacgccgaacatgatcgactatttcggacggccgtatgaaggcatcgccgtgttcgacggcaaaaagatcactgtaacagggaccctgtggaacggcaacaaaattattgacgaacggctcatcaatcccgatggctctctcctcttccgggtaa

SEQ ID NO: 54 - DNA, 54 bp, synthetic construct
  source 1..54: mol_type = other DNA; note = nucleotide sequence ending 2A peptide used in Examples
  CDS 1..54: protein_id = 55; translation = EGRGSLLTCGDVEENPGP
gagggcagaggaagtcttctaacatgcggtgacgtggaggagaatcccggccct

SEQ ID NO: 55 - protein, 18 aa, synthetic construct
EGRGSLLTCGDVEENPGP

SEQ ID NO: 56 - DNA, 591 bp, Corynebacterium diphtheriae
  source 1..591: mol_type = genomic DNA
  CDS 1..591: protein_id = 57; translation = MDPDDVVDSSKSFVMENFSSYHGTKPGYVDSIQKGIQKPKSGTQGNYDDDWKGFYSTDNKYDAAGYSVDNENPLSGKAGGVVKVTYPGLTKVLALKVDNAETIKKELGLSLTEPLMEQVGTEEFIKRFGDGASRVVLSLPFAEGSSSVEYINNWEQAKALSVELEINFETRGKRGQDAMYEYMAQACAGNRVRRSL
atggatcctgatgatgttgttgattcttctaaatcttttgtgatggaaaacttttcttcgtaccacgggactaaacctggttatgtagattccattcaaaaaggtatacaaaagccaaaatctggtacacaaggaaattatgacgatgattggaaagggttttatagtaccgacaataaatacgacgctgcgggatactctgtagataatgaaaacccgctctctggaaaagctggaggcgtggtcaaagtgacgtatccaggactgacgaaggttctcgcactaaaagtggataatgccgaaactattaagaaagagttaggtttaagtctcactgaaccgttgatggagcaagtcggaacggaagagtttatcaaaaggttcggtgatggtgcttcgcgtgtagtgctcagccttcccttcgctgaggggagttctagcgttgaatatattaataactgggaacaggcgaaagcgttaagcgtagaacttgagattaattttgaaacccgtggaaaacgtggccaagatgcgatgtatgagtatatggctcaagcctgtgcaggaaatcgtgtcaggcgatctttgtga

SEQ ID NO: 57 - protein, 196 aa, Corynebacterium diphtheriae
MDPDDVVDSSKSFVMENFSSYHGTKPGYVDSIQKGIQKPKSGTQGNYDDDWKGFYSTDNKYDAAGYSVDNENPLSGKAGGVVKVTYPGLTKVLALKVDNAETIKKELGLSLTEPLMEQVGTEEFIKRFGDGASRVVLSLPFAEGSSSVEYINNWEQAKALSVELEINFETRGKRGQDAMYEYMAQACAGNRVRRSL

SEQ ID NO: 58 - DNA, 1209 bp, synthetic construct
  source 1..1209: mol_type = other DNA; note = Nluc-2A-DTA fragment
  CDS 1..1209: protein_id = 59; translation = MVFTLEDFVGDWRQTAGYNLDQVLEQGGVSSLFQNLGVSVTPIQRIVLSGENGLKIDIHVIIPYEGLSGDQMGQIEKIFKVVYPVDDHHFKVILHYGTLVIDGVTPNMIDYFGRPYEGIAVFDGKKITVTGTLWNGNKIIDERLINPDGSLLFRVTINGVTGWRLCERILAITSYSIHYTKLFEGRGSLLTCGDVEENPGPRDPPVMDPDDVVDSSKSFVMENFSSYHGTKPGYVDSIQKGIQKPKSGTQGNYDDDWKGFYSTDNKYDAAGYSVDNENPLSGKAGGVVKVTYPGLTKVLALKVDNAETIKKELGLSLTEPLMEQVGTEEFIKRFGDGASRVVLSLPFAEGSSSVEYINNWEQAKALSVELEINFETRGKRGQDAMYEYMAQACAGNRVRRSL
atggtcttcacactcgaagatttcgttggggactggcgacagacagccggctacaacctggaccaagtccttgaacagggaggtgtgtccagtttgtttcagaatctcggggtgtccgtaactccgatccaaaggattgtcctgagcggtgaaaatgggctgaagatcgacatccatgtcatcatcccgtatgaaggtctgagcggcgaccaaatgggccagatcgaaaaaatttttaaggtggtgtaccctgtggatgatcatcactttaaggtgatcctgcactatggcacactggtaatcgacggggttacgccgaacatgatcgactatttcggacggccgtatgaaggcatcgccgtgttcgacggcaaaaagatcactgtaacagggaccctgtggaacggcaacaaaattatcgacgagcgcctgatcaaccccgacggctccctgctgttccgagtaaccatcaacggagtgaccggctggcggctgtgcgaacgcattctggcgataacttcgtatagcatacattatacgaagttatttgagggcagaggaagtcttctaacatgcggtgacgtggaggagaatcccggccctcgagatccaccggtcatggatcctgatgatgttgttgattcttctaaatcttttgtgatggaaaacttttcttcgtaccacgggactaaacctggttatgtagattccattcaaaaaggtatacaaaagccaaaatctggtacacaaggaaattatgacgatgattggaaagggttttatagtaccgacaataaatacgacgctgcgggatactctgtagataatgaaaacccgctctctggaaaagctggaggcgtggtcaaagtgacgtatccaggactgacgaaggttctcgcactaaaagtggataatgccgaaactattaagaaagagttaggtttaagtctcactgaaccgttgatggagcaagtcggaacggaagagtttatcaaaaggttcggtgatggtgcttcgcgtgtagtgctcagccttcccttcgctgaggggagttctagcgttgaatatattaataactgggaacaggcgaaagcgttaagcgtagaacttgagattaattttgaaacccgtggaaaacgtggccaagatgcgatgtatgagtatatggctcaagcctgtgcaggaaatcgtgtcaggcgatctttgtga

SEQ ID NO: 59 - protein, 402 aa, synthetic construct
MVFTLEDFVGDWRQTAGYNLDQVLEQGGVSSLFQNLGVSVTPIQRIVLSGENGLKIDIHVIIPYEGLSGDQMGQIEKIFKVVYPVDDHHFKVILHYGTLVIDGVTPNMIDYFGRPYEGIAVFDGKKITVTGTLWNGNKIIDERLINPDGSLLFRVTINGVTGWRLCERILAITSYSIHYTKLFEGRGSLLTCGDVEENPGPRDPPVMDPDDVVDSSKSFVMENFSSYHGTKPGYVDSIQKGIQKPKSGTQGNYDDDWKGFYSTDNKYDAAGYSVDNENPLSGKAGGVVKVTYPGLTKVLALKVDNAETIKKELGLSLTEPLMEQVGTEEFIKRFGDGASRVVLSLPFAEGSSSVEYINNWEQAKALSVELEINFETRGKRGQDAMYEYMAQACAGNRVRRSL

SEQ ID NO: 60 - DNA, 1209 bp, synthetic construct
  source 1..1209: mol_type = other DNA; note = SceNluc-2A-DTA fragment
  CDS 1..225: protein_id = 61; translation = MVFTLEDFVGDWRQTAGYNLDQVLEQGGVSSLFQNLGVSVTPIQRIVLSGENGLKIDIHVIIPYEGLSGDQMGQ
  CDS 235..1209: protein_id = 62; translation = QGNVYPVDDHHFKVILHYGTLVIDGVTPNMIDYFGRPYEGIAVFDGKKITVTGTLWNGNKIIDERLINPDGSLLFRVTINGVTGWRLCERILAITSYSIHYTKLFEGRGSLLTCGDVEENPGPRDPPVMDPDDVVDSSKSFVMENFSSYHGTKPGYVDSIQKGIQKPKSGTQGNYDDDWKGFYSTDNKYDAAGYSVDNENPLSGKAGGVVKVTYPGLTKVLALKVDNAETIKKELGLSLTEPLMEQVGTEEFIKRFGDGASRVVLSLPFAEGSSSVEYINNWEQAKALSVELEINFETRGKRGQDAMYEYMAQACAGNRVRRSL
atggtcttcacactcgaagatttcgttggggactggcgacagacagccggctacaacctggaccaagtccttgaacagggaggtgtgtccagtttgtttcagaatctcggggtgtccgtaactccgatccaaaggattgtcctgagcggtgaaaatgggctgaagatcgacatccatgtcatcatcccgtatgaaggtctgagcggcgaccaaatgggccagtgatagggataacagggtaatgtgtaccctgtggatgatcatcactttaaggtgatcctgcactatggcacactggtaatcgacggggttacgccgaacatgatcgactatttcggacggccgtatgaaggcatcgccgtgttcgacggcaaaaagatcactgtaacagggaccctgtggaacggcaacaaaattatcgacgagcgcctgatcaaccccgacggctccctgctgttccgagtaaccatcaacggagtgaccggctggcggctgtgcgaacgcattctggcgataacttcgtatagcatacattatacgaagttatttgagggcagaggaagtcttctaacatgcggtgacgtggaggagaatcccggccctcgagatccaccggtcatggatcctgatgatgttgttgattcttctaaatcttttgtgatggaaaacttttcttcgtaccacgggactaaacctggttatgtagattccattcaaaaaggtatacaaaagccaaaatctggtacacaaggaaattatgacgatgattggaaagggttttatagtaccgacaataaatacgacgctgcgggatactctgtagataatgaaaacccgctctctggaaaagctggaggcgtggtcaaagtgacgtatccaggactgacgaaggttctcgcactaaaagtggataatgccgaaactattaagaaagagttaggtttaagtctcactgaaccgttgatggagcaagtcggaacggaagagtttatcaaaaggttcggtgatggtgcttcgcgtgtagtgctcagccttcccttcgctgaggggagttctagcgttgaatatattaataactgggaacaggcgaaagcgttaagcgtagaacttgagattaattttgaaacccgtggaaaacgtggccaagatgcgatgtatgagtatatggctcaagcctgtgcaggaaatcgtgtcaggcgatctttgtga

SEQ ID NO: 61 - protein, 74 aa, synthetic construct; identical to SEQ ID NO: 10

SEQ ID NO: 62 - protein, 324 aa, synthetic construct
QGNVYPVDDHHFKVILHYGTLVIDGVTPNMIDYFGRPYEGIAVFDGKKITVTGTLWNGNKIIDERLINPDGSLLFRVTINGVTGWRLCERILAITSYSIHYTKLFEGRGSLLTCGDVEENPGPRDPPVMDPDDVVDSSKSFVMENFSSYHGTKPGYVDSIQKGIQKPKSGTQGNYDDDWKGFYSTDNKYDAAGYSVDNENPLSGKAGGVVKVTYPGLTKVLALKVDNAETIKKELGLSLTEPLMEQVGTEEFIKRFGDGASRVVLSLPFAEGSSSVEYINNWEQAKALSVELEINFETRGKRGQDAMYEYMAQACAGNRVRRSL

SEQ ID NO: 63 - DNA, 1131 bp, Human alphaherpesvirus 1
  source 1..1131: mol_type = genomic DNA
  CDS 1..1131: protein_id = 64; translation = MASYPGHQHASAFDQAARSRGHSNRRTALRPRRQQEATEVRPEQKMPTLLRVYIDGPHGMGKTTTTQLLVALGSRDDIVYVPEPMTYWRVLGASETIANIYTTQHRLDQGEISAGDAAVVMTSAQITMGMPYAVTDAVLAPHIGGEAGSSHAPPPALTLIFDRHPIAALLCYPAARYLMGSMTPQAVLAFVALIPPTLPGTNIVLGALPEDRHIDRLAKRQRPGERLDLAMLAAIRRVYGLLANTVRYLQCGGSWREDWGQLSGTAVPPQGAEPQSNAGPRPHIGDTLFTLFRAPELLAPNGDLYNVFAWALDVLAKRLRSMHVFILDYDQSPAGCRDALLQLTSGMVQTHVTTPGSIPTICDLARTFAREMGEAN
atggcttcgtaccccggccatcaacacgcgtctgcgttcgaccaggctgcgcgttctcgcggccatagcaaccgacgtacggcgttgcgccctcgccggcagcaagaagccacggaagtccgcccggagcagaaaatgcccacgctactgcgggtttatatagacggtccccacgggatggggaaaaccaccaccacgcaactgctggtggccctgggttcgcgcgacgatatcgtctacgtacccgagccgatgacttactggcgggtgctgggggcttccgagacaatcgcgaacatctacaccacacaacaccgcctcgaccagggtgagatatcggccggggacgcggcggtggtaatgacaagcgcccagataacaatgggcatgccttatgccgtgaccgacgccgttctggctcctcatatcgggggggaggctgggagctcacatgccccgcccccggccctcaccctcatcttcgaccgccatcccatcgccgccctcctgtgctacccggccgcgcggtaccttatgggcagcatgaccccccaggccgtgctggcgttcgtggccctcatcccgccgaccttgcccggcaccaacatcgtgcttggggcccttccggaggacagacacatcgaccgcctggccaaacgccagcgccccggcgagcggctggacctggctatgctggctgcgattcgccgcgtttacgggctacttgccaatacggtgcggtatctgcagtgcggcgggtcgtggcgggaggactggggacagctttcggggacggccgtgccgccccagggtgccgagccccagagcaacgcgggcccacgaccccatatcggggacacgttatttaccctgtttcgggcccccgagttgctggcccccaacggcgacctgtataacgtgtttgcctgggccttggacgtcttggccaaacgcctccgttccatgcacgtctttatcctggattacgaccaatcgcccgccggctgccgggacgccctgctgcaacttacctccgggatggtccagacccacgtcaccacccccggctccataccgacgatatgcgacctggcgcgcacgtttgcccgggagatgggggaggctaactga

SEQ ID NO: 64 - protein, 376 aa, Human alphaherpesvirus 1
MASYPGHQHASAFDQAARSRGHSNRRTALRPRRQQEATEVRPEQKMPTLLRVYIDGPHGMGKTTTTQLLVALGSRDDIVYVPEPMTYWRVLGASETIANIYTTQHRLDQGEISAGDAAVVMTSAQITMGMPYAVTDAVLAPHIGGEAGSSHAPPPALTLIFDRHPIAALLCYPAARYLMGSMTPQAVLAFVALIPPTLPGTNIVLGALPEDRHIDRLAKRQRPGERLDLAMLAAIRRVYGLLANTVRYLQCGGSWREDWGQLSGTAVPPQGAEPQSNAGPRPHIGDTLFTLFRAPELLAPNGDLYNVFAWALDVLAKRLRSMHVFILDYDQSPAGCRDALLQLTSGMVQTHVTTPGSIPTICDLARTFAREMGEAN

SEQ ID NO: 65 - DNA, 63 bp, synthetic construct
  source 1..63: mol_type = other DNA; note = primer TK-Fw
taatacgactcactataggctagcctcgagatccaccggtcatggcttcgtaccccggccatc

SEQ ID NO: 66 - DNA, 45 bp, synthetic construct
  source 1..45: mol_type = other DNA; note = primer TK-Rv
ccgccccgactctagagtcgcggtcagttagcctcccccatctcc

SEQ ID NO: 67 - DNA, 1749 bp, synthetic construct
  source 1..1749: mol_type = other DNA; note = SceNluc-2A-TK fragment
  CDS 1..225: protein_id = 68; translation = MVFTLEDFVGDWRQTAGYNLDQVLEQGGVSSLFQNLGVSVTPIQRIVLSGENGLKIDIHVIIPYEGLSGDQMGQ
  CDS 235..1749: protein_id = 69; translation = QGNVYPVDDHHFKVILHYGTLVIDGVTPNMIDYFGRPYEGIAVFDGKKITVTGTLWNGNKIIDERLINPDGSLLFRVTINGVTGWRLCERILAITSYSIHYTKLFEGRGSLLTCGDVEENPGPRDPPVMASYPGHQHASAFDQAARSRGHSNRRTALRPRRQQEATEVRPEQKMPTLLRVYIDGPHGMGKTTTTQLLVALGSRDDIVYVPEPMTYWRVLGASETIANIYTTQHRLDQGEISAGDAAVVMTSAQITMGMPYAVTDAVLAPHIGGEAGSSHAPPPALTLIFDRHPIAALLCYPAARYLMGSMTPQAVLAFVALIPPTLPGTNIVLGALPEDRHIDRLAKRQRPGERLDLAMLAAIRRVYGLLANTVRYLQCGGSWREDWGQLSGTAVPPQGAEPQSNAGPRPHIGDTLFTLFRAPELLAPNGDLYNVFAWALDVLAKRLRSMHVFILDYDQSPAGCRDALLQLTSGMVQTHVTTPGSIPTICDLARTFAREMGEAN
atggtcttcacactcgaagatttcgttggggactggcgacagacagccggctacaacctggaccaagtccttgaacagggaggtgtgtccagtttgtttcagaatctcggggtgtccgtaactccgatccaaaggattgtcctgagcggtgaaaatgggctgaagatcgacatccatgtcatcatcccgtatgaaggtctgagcggcgaccaaatgggccagtgatagggataacagggtaatgtgtaccctgtggatgatcatcactttaaggtgatcctgcactatggcacactggtaatcgacggggttacgccgaacatgatcgactatttcggacggccgtatgaaggcatcgccgtgttcgacggcaaaaagatcactgtaacagggaccctgtggaacggcaacaaaattatcgacgagcgcctgatcaaccccgacggctccctgctgttccgagtaaccatcaacggagtgaccggctggcggctgtgcgaacgcattctggcgataacttcgtatagcatacattatacgaagttatttgagggcagaggaagtcttctaacatgcggtgacgtggaggagaatcccggccctcgagatccaccggtcatggcttcgtaccccggccatcaacacgcgtctgcgttcgaccaggctgcgcgttctcgcggccatagcaaccgacgtacggcgttgcgccctcgccggcagcaagaagccacggaagtccgcccggagcagaaaatgcccacgctactgcgggtttatatagacggtccccacgggatggggaaaaccaccaccacgcaactgctggtggccctgggttcgcgcgacgatatcgtctacgtacccgagccgatgacttactggcgggtgctgggggcttccgagacaatcgcgaacatctacaccacacaacaccgcctcgaccagggtgagatatcggccggggacgcggcggtggtaatgacaagcgcccagataacaatgggcatgccttatgccgtgaccgacgccgttctggctcctcatatcgggggggaggctgggagctcacatgccccgcccccggccctcaccctcatcttcgaccgccatcccatcgccgccctcctgtgctacccggccgcgcggtaccttatgggcagcatgaccccccaggccgtgctggcgttcgtggccctcatcccgccgaccttgcccggcaccaacatcgtgcttggggcccttccggaggacagacacatcgaccgcctggccaaacgccagcgccccggcgagcggctggacctggctatgctggctgcgattcgccgcgtttacgggctacttgccaatacggtgcggtatctgcagtgcggcgggtcgtggcgggaggactggggacagctttcggggacggccgtgccgccccagggtgccgagccccagagcaacgcgggcccacgaccccatatcggggacacgttatttaccctgtttcgggcccccgagttgctggcccccaacggcgacctgtataacgtgtttgcctgggccttggacgtcttggccaaacgcctccgttccatgcacgtctttatcctggattacgaccaatcgcccgccggctgccgggacgccctgctgcaacttacctccgggatggtccagacccacgtcaccacccccggctccataccgacgatatgcgacctggcgcgcacgtttgcccgggagatgggggaggctaactga

SEQ ID NO: 68 - protein, 74 aa, synthetic construct; identical to SEQ ID NO: 10

SEQ ID NO: 69 - protein, 504 aa, synthetic construct
QGNVYPVDDHHFKVILHYGTLVIDGVTPNMIDYFGRPYEGIAVFDGKKITVTGTLWNGNKIIDERLINPDGSLLFRVTINGVTGWRLCERILAITSYSIHYTKLFEGRGSLLTCGDVEENPGPRDPPVMASYPGHQHASAFDQAARSRGHSNRRTALRPRRQQEATEVRPEQKMPTLLRVYIDGPHGMGKTTTTQLLVALGSRDDIVYVPEPMTYWRVLGASETIANIYTTQHRLDQGEISAGDAAVVMTSAQITMGMPYAVTDAVLAPHIGGEAGSSHAPPPALTLIFDRHPIAALLCYPAARYLMGSMTPQAVLAFVALIPPTLPGTNIVLGALPEDRHIDRLAKRQRPGERLDLAMLAAIRRVYGLLANTVRYLQCGGSWREDWGQLSGTAVPPQGAEPQSNAGPRPHIGDTLFTLFRAPELLAPNGDLYNVFAWALDVLAKRLRSMHVFILDYDQSPAGCRDALLQLTSGMVQTHVTTPGSIPTICDLARTFAREMGEAN

SEQ ID NO: 70 - DNA, 45 bp, synthetic construct
  source 1..45: mol_type = other DNA; note = primer DTA-Fw
actcactataggctagcgtcctcgccatggatcctgatgatgttg

SEQ ID NO: 71 - DNA, 40 bp, synthetic construct
  source 1..40: mol_type = other DNA; note = primer Sce-5'DTA-Rv
attaccctgttatccctatcattgtgtaccagattttggc

SEQ ID NO: 72 - DNA, 41 bp, synthetic construct
  source 1..41: mol_type = other DNA; note = primer Sce-3'DTA-Fw
tagggataacagggtaataaagggttttatagtaccgacaa

SEQ ID NO: 73 - DNA, 46 bp, synthetic construct
  source 1..46: mol_type = other DNA; note = primer DTA-Rv
ccgccccgactctagaatcacaaagatcgcctgacacgatttcctg

SEQ ID NO: 74 - DNA, 28 bp, synthetic construct
  source 1..28: mol_type = other DNA; note = primer iDTA2-Fw
atcttttgtgatggaaaacttttcttcg

SEQ ID NO: 75 - DNA, 22 bp, synthetic construct
  source 1..22: mol_type = other DNA; note = primer iDTA2-Rv
tcactttgaccacgcctccagc

SEQ ID NO: 76 - DNA, 591 bp, synthetic construct
  source 1..591: mol_type = other DNA; note = SceDTA gene
  CDS 1..135: protein_id = 77; translation = MDPDDVVDSSKSFVMENFSSYHGTKPGYVDSIQKGIQKPKSGTQ
  CDS 145..591: protein_id = 78; translation = QGNKGFYSTDNKYDAAGYSVDNENPLSGKAGGVVKVTYPGLTKVLALKVDNAETIKKELGLSLTEPLMEQVGTEEFIKRFGDGASRVVLSLPFAEGSSSVEYINNWEQAKALSVELEINFETRGKRGQDAMYEYMAQACAGNRVRRSL
atggatcctgatgatgttgttgattcttctaaatcttttgtgatggaaaacttttcttcgtaccacgggactaaacctggttatgtagattccattcaaaaaggtatacaaaagccaaaatctggtacacaatgatagggataacagggtaataaagggttttatagtaccgacaataaatacgacgctgcgggatactctgtagataatgaaaacccgctctctggaaaagctggaggcgtggtcaaagtgacgtatccaggactgacgaaggttctcgcactaaaagtggataatgccgaaactattaagaaagagttaggtttaagtctcactgaaccgttgatggagcaagtcggaacggaagagtttatcaaaaggttcggtgatggtgcttcgcgtgtagtgctcagccttcccttcgctgaggggagttctagcgttgaatatattaataactgggaacaggcgaaagcgttaagcgtagaacttgagattaattttgaaacccgtggaaaacgtggccaagatgcgatgtatgagtatatggctcaagcctgtgcaggaaatcgtgtcaggcgatctttgtga

SEQ ID NO: 77 - protein, 44 aa, synthetic construct
MDPDDVVDSSKSFVMENFSSYHGTKPGYVDSIQKGIQKPKSGTQ

SEQ ID NO: 78 - protein, 148 aa, synthetic construct
QGNKGFYSTDNKYDAAGYSVDNENPLSGKAGGVVKVTYPGLTKVLALKVDNAETIKKELGLSLTEPLMEQVGTEEFIKRFGDGASRVVLSLPFAEGSSSVEYINNWEQAKALSVELEINFETRGKRGQDAMYEYMAQACAGNRVRRSL

SEQ ID NO: 79 - DNA, 221 bp, synthetic construct
  source 1..221: mol_type = other DNA; note = iDTA2 gene (homology 100%)
  CDS 2..221: protein_id = 80; translation = SFVMENFSSYHGTKPGYVDSIQKGIQKPKSGTQGNYDDDWKGFYSTDNKYDAAGYSVDNENPLSGKAGGVVKV
atcttttgtgatggaaaacttttcttcgtaccacgggactaaacctggttatgtagattccattcaaaaaggtatacaaaagccaaaatctggtacacaaggaaattatgacgatgattggaaagggttttatagtaccgacaataaatacgacgctgcgggatactctgtagataatgaaaacccgctctctggaaaagctggaggcgtggtcaaagtga

SEQ ID NO: 80 - protein, 73 aa, synthetic construct
SFVMENFSSYHGTKPGYVDSIQKGIQKPKSGTQGNYDDDWKGFYSTDNKYDAAGYSVDNENPLSGKAGGVVKV

SEQ ID NO: 81 - DNA, 221 bp, synthetic construct
  source 1..221: mol_type = other DNA; note = iDTA2 gene (homology 99%)
atcttttgtgatggaaaacttttcttcgtaccacgggactaaacctggttacgtagattccattcaaaaaggtatacaaaagccaaaatctggtacacaaggaaattatgacgatgattggaaagggttttatagtaccgacaataaatacgacgctgcgggatactctgtggataatgaaaacccgctctctggaaaagctggaggcgtggtcaaagtga

SEQ ID NO: 82 - DNA, 221 bp, synthetic construct
  source 1..221: mol_type = other DNA; note = iDTA2 gene (homology 98%)
atcttttgtgatggaaaacttttcttcgtaccatgggactaaacctggttatgtagattccattcagaaaggtatacaaaagccaaaatctggtacacaaggaaattatgacgatgattggaaagggttttatagtaccgacaataaatacgatgctgcgggatactctgtagataatgaaaaccccctctctggaaaagctggaggcgtggtcaaagtga

SEQ ID NO: 83 - DNA, 221 bp, synthetic construct
  source 1..221: mol_type = other DNA; note = iDTA2 gene (homology 97%)
atcttttgtgatggaaaacttttcttcctaccacgggactaaacctggttacgtagattccattcaaaaaggtatccaaaagccaaaatctggtacacaaggaaattatgacgatgattggaaagggttttatagtaccgacaacaaatacgacgctgcgggatactccgtagataatgaaaacccgctctccggaaaagctggaggcgtggtcaaagtga

SEQ ID NO: 84 - DNA, 221 bp, synthetic construct
  source 1..221: mol_type = other DNA; note = iDTA2 gene (homology 96%)
atcttttgtgatggaaaacttctcttcgtaccacgggaccaaacctggttatgtagactctattcaaaaaggtatacagaagccaaaatctggtacacaaggaaattatgacgatgattggaaagggttttatagtaccgataataaatacgacgctgcaggatactctgtagataatgagaacccgctctctggaaaggctggaggcgtggtcaaagtga

SEQ ID NO: 85 - DNA, 221 bp, synthetic construct
  source 1..221: mol_type = other DNA; note = iDTA2 gene (homology 95%)
atcttttgtgatggaaaatttttcttcgtaccatgggactaaacctggctatgtagattccatccaaaaaggtatacaaaaaccaaaatctggtacacaaggaaattatgacgatgattggaaagggttttatagtacagacaataaatacgacgccgcgggatactctgtggataatgaaaaccccctctctggaaaagccggaggcgtggtcaaagtga

SEQ ID NO: 86 - DNA, 221 bp, synthetic construct
  source 1..221: mol_type = other DNA; note = iDTA2 gene (homology 94%)
atcttttgtgatggagaacttttcttcgtatcacgggactaagcctggttatgtagactccattcaaaagggtatacaaaagcccaaatctggtacacaaggaaattatgacgatgattggaaagggttttatagcaccgacaataaatatgacgctgcgggctactctgtagataacgaaaacccgctgtctggaaaagctggcggcgtggtcaaagtga

SEQ ID NO: 87 - DNA, 221 bp, synthetic construct
  source 1..221: mol_type = other DNA; note = iDTA2 gene (homology 90%)
atcttttgtcatggaaaatttttcttcctaccacggcactaaacccggttatgtggattccatccaaaaaggcatacaaaaaccaaaatccggtacacaaggaaattatgacgatgattggaaagggttctatagtacagacaataagtacgacgccgcgggatattctgtagacaatgaaaatccgctctccggaaaagccggaggcgtcgtcaaagtga

SEQ ID NO: 88 - DNA, 221 bp, synthetic construct
  source 1..221: mol_type = other DNA; note = iDTA2 gene (homology 80%)
atcctttgtcatggagaacttctcctcctaccatgggaccaagcccggttacgtagactctatccaaaagggtatccagaaaccaaagtctggcacacaaggaaattatgacgatgattggaaaggcttttacagtacagataacaaatatgacgccgcaggctactccgtagacaacgagaaccccctctccggcaaggctggcggcgtcgtcaaggtga

SEQ ID NO: 89 - DNA, 221 bp, synthetic construct
  source 1..221: mol_type = other DNA; note = iDTA2 gene (homology 70%)
atccttcgtcatggagaatttctcctcctatcatggcaccaagcccggctacgtggactctatccagaagggcatccagaaacccaagtccggcacccaaggaaattatgacgatgattggaaaggcttctacagcacagataacaagtatgatgccgcaggctattccgtggacaacgagaatcccctgtccggcaaggccggcggggtcgtgaaggtga

SEQ ID NO: 90 - DNA, 50 bp, synthetic construct
  source 1..50: mol_type = other DNA; note = primer 5'SceDTA3-Rv
cattaccctgttatccctacgcgtcacagtgtaccagattttggcttttg

SEQ ID NO: 91 - DNA, 46 bp, synthetic construct
  source 1..46: mol_type = other DNA; note = primer 3'SceDTA3-Fw
gtagggataacagggtaatgcatacaggcgaaagcgttaagcgtag

SEQ ID NO: 92 - DNA, 29 bp, synthetic construct
  source 1..29: mol_type = other DNA; note = primer iDTA3-1-100-Fw
ttatgtagattccattcaaaaaggtatac

SEQ ID NO: 93 - DNA, 27 bp, synthetic construct
  source 1..27: mol_type = other DNA; note = primer iDTA3-1-100-Rv
gacttaaacctaactctttcttaatag

SEQ ID NO: 94 - DNA, 23 bp, synthetic construct
  source 1..23: mol_type = other DNA; note = primer iDTA3-2-100-Fw
gctggaggcgtggtcaaagtgac

SEQ ID NO: 95 - DNA, 25 bp, synthetic construct
  source 1..25: mol_type = other DNA; note = primer iDTA3-2-100-Rv
cacgggtttcaaaattaatctcaag

SEQ ID NO: 96 - DNA, 35 bp, synthetic construct
  source 1..35: mol_type = other DNA; note = primer iDTA3-1-98-Fw
ttatgtagattccattcaaaaaggcatacaaaagc

SEQ ID NO: 97 - DNA, 43 bp, synthetic construct
  source 1..43: mol_type = other DNA; note = primer iDTA3-1-98-Rv
gacttaaacctaactctttcttaatagtttcggcgttatccac

SEQ ID NO: 98 - DNA, 45 bp, synthetic construct
  source 1..45: mol_type = other DNA; note = primer iDTA3-1-94-Fw
ttatgtagattctattcaaaaaggcatacaaaagcccaaatctgg

SEQ ID NO: 99 - DNA, 52 bp, synthetic construct
  source 1..52: mol_type = other DNA; note = primer iDTA3-1-94-Rv
gacttaaacctaactccttcttaatagtttcagcattatccacctttagtgc

SEQ ID NO: 100 - DNA, 48 bp, synthetic construct
  source 1..48: mol_type = other DNA; note = primer iDTA3-1-90-Fw
ttatgtcgattccatccaaaaaggcatacaaaaaccaaaatccggtac

SEQ ID NO: 101 - DNA, 52 bp, synthetic construct
  source 1..52: mol_type = other DNA; note = primer iDTA3-1-90-Rv
gacttaagcctaactccttcttaatggtttcggcgttatccacctttagtgc

SEQ ID NO: 102 - DNA, 39 bp, synthetic construct
  source 1..39: mol_type = other DNA; note = primer iDTA3-2-98-Fw
gctggaggcgtggtcaaagtgacgtatccagggctgacg

SEQ ID NO: 103 - DNA, 32 bp, synthetic construct
  source 1..32: mol_type = other DNA; note = primer iDTA3-2-98-Rv
cacgggtttcaaaattaatctcaagctctacg

SEQ ID NO: 104 - DNA, 49 bp, synthetic construct
  source 1..49: mol_type = other DNA; note = primer iDTA3-2-94-Fw
gctggaggcgtggtgaaagtgacgtatcccggactgacgaaagttctcg

SEQ ID NO: 105 - DNA, 45 bp, synthetic construct
  source 1..45: mol_type = other DNA; note = primer iDTA3-2-94-Rv
cacgggtttcaaagttaatctcaagctctacgcttaaggctttcg

SEQ ID NO: 106 - DNA, 52 bp, synthetic construct
  source 1..52: mol_type = other DNA; note = primer iDTA3-2-90-Fw
gctggaggcgtcgtcaaagtcacgtatcccggactgaccaaggttctggcac

SEQ ID NO: 107 - DNA, 49 bp, synthetic construct
  source 1..49: mol_type = other DNA; note = primer iDTA3-2-90-Rv
cacgggtctcaaaattgatctcaagctctacgctcaacgctttggcctg

SEQ ID NO: 108 - DNA, 288 bp, synthetic construct
  source 1..288: mol_type = other DNA
  CDS 1..135: protein_id = 109; translation = MDPDDVVDSSKSFVMENFSSYHGTKPGYVDSIQKGIQKPKSGTL
  CDS 136..156: protein_id = 110; translation = RVGITG
  CDS 157..288: protein_id = 111; translation = CIQAKALSVELEINFETRGKRGQDAMYEYMAQACAGNRVRRSL
atggatcctgatgatgttgttgattcttctaaatcttttgtgatggaaaacttttcttcgtaccacgggactaaacctggttatgtagattccattcaaaaaggtatacaaaagccaaaatctggtacactgtgacgcgtagggataacagggtaatgcatacaggcgaaagcgttaagcgtagaacttgagattaattttgaaacccgtggaaaacgtggccaagatgcgatgtatgagtatatggctcaagcctgtgcaggaaatcgtgtcaggcgatctttgtga

SEQ ID NO: 109 - protein, 44 aa, synthetic construct
MDPDDVVDSSKSFVMENFSSYHGTKPGYVDSIQKGIQKPKSGTL

SEQ ID NO: 110 - protein, 6 aa, synthetic construct
RVGITG

SEQ ID NO: 111 - protein, 43 aa, synthetic construct
CIQAKALSVELEINFETRGKRGQDAMYEYMAQACAGNRVRRSL

SEQ ID NO: 112 - DNA, 251 bp, synthetic construct
  source 1..251: mol_type = other DNA; note = iDTA3-1-100 gene
ttatgtagattccattcaaaaaggtatacaaaagccaaaatctggtacacaaggaaattatgacgatgattggaaagggttttatagtaccgacaataaatacgacgctgcgggatactctgtagataatgaaaacccgctctctggaaaagctggaggcgtggtcaaagtgacgtatccaggactgacgaaggttctcgcactaaaagtggataatgccgaaactattaagaaagagttaggtttaagtc

SEQ ID NO: 113 - DNA, 283 bp, synthetic construct
  source 1..283: mol_type = other DNA; note = iDTA3-2-100 gene
gctggaggcgtggtcaaagtgacgtatccaggactgacgaaggttctcgcactaaaagtggataatgccgaaactattaagaaagagttaggtttaagtctcactgaaccgttgatggagcaagtcggaacggaagagtttatcaaaaggttcggtgatggtgcttcgcgtgtagtgctcagccttcccttcgctgaggggagttctagcgttgaatatattaataactgggaacaggcgaaagcgttaagcgtagaacttgagattaattttgaaacccgtg

SEQ ID NO: 114 - DNA, 251 bp, synthetic construct
  source 1..251: mol_type = other DNA; note = iDTA3-1-98 gene
ttatgtagattccattcaaaaaggcatacaaaagccaaaatctggtacacaaggaaattatgacgatgattggaaagggttttatagtaccgacaataaatacgacgctgcgggatactctgtagataatgaaaacccgctctctggaaaagctggaggcgtggtcaaagtgacgtatccaggactgacgaaggttctcgcactaaaagtggataacgccgaaactattaagaaagagttaggtttaagtc

SEQ ID NO: 115 - DNA, 251 bp, synthetic construct
  source 1..251: mol_type = other DNA; note = iDTA3-1-94 gene
ttatgtagattctattcaaaaaggcatacaaaagcccaaatctggtacacaaggaaattatgacgatgattggaaagggttttatagtaccgacaataaatacgacgctgcgggatactctgtagataatgaaaacccgctctctggaaaagctggaggcgtggtcaaagtgacgtatccaggactgacgaaggttctcgcactaaaggtggataatgctgaaactattaagaaggagttaggtttaagtc

SEQ ID NO: 116 - DNA, 251 bp, synthetic construct
  source 1..251: mol_type = other DNA; note = iDTA3-1-90 gene
ttatgtcgattccatccaaaaaggcatacaaaaaccaaaatccggtacacaaggaaattatgacgatgattggaaagggttttatagtaccgacaataaatacgacgctgcgggatactctgtagataatgaaaacccgctctctggaaaagctggaggcgtggtcaaagtgacgtatccaggactgacgaaggttctggcactaaaggtggataacgccgaaaccattaagaaggagttaggcttaagtc

SEQ ID NO: 117 - DNA, 283 bp, synthetic construct
  source 1..283: mol_type = other DNA; note = iDTA3-2-98 gene
gctggaggcgtggtcaaagtgacgtatccagggctgacgaaggttctcgcactaaaagtggataatgccgaaactattaagaaagagttaggtttaagtctcactgaaccgttgatggagcaagtcggaacggaagagtttatcaaaaggttcggtgatggtgcttcgcgtgtagtgctcagccttcccttcgctgaggggagttctagcgttgaatatattaataactgggaacaggcgaaagcgttaagcgtagagcttgagattaattttgaaacccgtg

SEQ ID NO: 118 - DNA, 283 bp, synthetic construct
  source 1..283: mol_type = other DNA; note = iDTA3-2-94 gene
gctggaggcgtggtgaaagtgacgtatcccggactgacgaaagttctcgcactaaaagtggataatgccgaaactattaagaaagagttaggtttaagtctcactgaaccgttgatggagcaagtcggaacggaagagtttatcaaaaggttcggtgatggtgcttcgcgtgtagtgctcagccttcccttcgctgaggggagttctagcgttgaatatattaataactgggaacaggcgaaagccttaagcgtagagcttgagattaactttgaaacccgtg

SEQ ID NO: 119 - DNA, 283 bp, synthetic construct
  source 1..283: mol_type = other DNA; note = iDTA3-2-90 gene
gctggaggcgtcgtcaaagtcacgtatcccggactgaccaaggttctggcactaaaagtggataatgccgaaactattaagaaagagttaggtttaagtctcactgaaccgttgatggagcaagtcggaacggaagagtttatcaaaaggttcggtgatggtgcttcgcgtgtagtgctcagccttcccttcgctgaggggagttctagcgttgaatatattaataactgggaacaggccaaagcgttgagcgtagagcttgagatcaattttgagacccgtg

SEQ ID NO: 120 - DNA, 26 bp, synthetic construct
  source 1..26: mol_type = other DNA; note = primer Sce-5'TK-Fw
cttaatacgactcactataggctagc

SEQ ID NO: 121 - DNA, 50 bp, synthetic construct
  source 1..50: mol_type = other DNA; note = primer 5'SceTK3-Rv
cattaccctgttatccctacgcgtcactttttctgctccgggcggacttc

SEQ ID NO: 122 - DNA, 46 bp, synthetic construct
  source 1..46: mol_type = other DNA; note = primer 3'SceTK3-Fw
gtagggataacagggtaatgcatcgtctttatcctggattacgacc

SEQ ID NO: 123 - DNA, 20 bp, synthetic construct
  source 1..20: mol_type = other DNA; note = primer Sce-3'TK-Rv
gagtgcaccatacgcggatc

SEQ ID NO: 124 - DNA, 23 bp, synthetic construct
  source 1..23: mol_type = other DNA; note = primer iTK3-1-100-Fw
gcgccctcgccggcagcaagaag

SEQ ID NO: 125 - DNA, 25 bp, synthetic construct
  source 1..25: mol_type = other DNA; note = primer iTK3-1-100-Rv
agctcccagcctcccccccgatatg

SEQ ID NO: 126 - DNA, 22 bp, synthetic construct
  source 1..22: mol_type = other DNA; note = primer iTK3-2-100-Fw
gcggcggtggtaatgacaagcg

SEQ ID NO: 127 - DNA, 22 bp, synthetic construct
  source 1..22: mol_type = other DNA; note = primer iTK3-2-100-Rv
acccgccgcactgcagataccg

SEQ ID NO: 128 - DNA, 23 bp, synthetic construct
  source 1..23: mol_type = other DNA; note = primer iTK3-3-100-Fw
cagcgccccggcgagcggctgga

SEQ ID NO: 129 - DNA, 22 bp, synthetic construct
  source 1..22: mol_type = other DNA; note = primer iTK3-3-100-Rv
gggcgtcccggcagccggcggg

SEQ ID NO: 130 - DNA, 32 bp, synthetic construct
  source 1..32: mol_type = other DNA; note = primer iTK3-1-98-Fw
gcgccctcgccggcagcaagaagctacggaag

SEQ ID NO: 131 - DNA, 40 bp, synthetic construct
  source 1..40: mol_type = other DNA; note = primer iTK3-1-98-Rv
agctcccagcctcccccccgatatgaggagccagcacggc

SEQ ID NO: 132 - DNA, 43 bp, synthetic construct
  source 1..43: mol_type = other DNA; note = primer iTK3-1-94-Fw
gcgccctcgccgccagcaagaagctacggaagtccggccggag

SEQ ID NO: 133 - DNA, 50 bp, synthetic construct
  source 1..50: mol_type = other DNA; note = primer iTK3-1-94-Rv
agctcccagcctccccgccgatatgaggggccagaacggcgtctgtcacg

SEQ ID NO: 134 - DNA, 48 bp, synthetic construct
  source 1..48: mol_type = other DNA; note = primer iTK3-1-90-Fw
gcgcccccgccggcaacaagaagctacggaagtgcgcccggaacagaa

SEQ ID NO: 135 - DNA, 50 bp, synthetic construct
  source 1..50: mol_type = other DNA; note = primer iTK3-1-90-Rv
agctcccggcctccccgccgatatggggagccagcacggcgtctgtcacg

SEQ ID NO: 136 - DNA, 38 bp, synthetic construct
  source 1..38: mol_type = other DNA; note = primer iTK3-2-98-Fw
gcggcggtggtaatgacaagcgcccagataaccatggg

SEQ ID NO: 137 - DNA, 41 bp, synthetic construct
  source 1..41: mol_type = other DNA; note = primer iTK3-2-98-Rv
acccgccgcactgcagataccgcaccgtattagcaagtagc

SEQ ID NO: 138 - DNA, 51 bp, synthetic construct
  source 1..51: mol_type = other DNA; note = primer iTK3-2-94-Fw
gcggcggtggtaatgaccagcgcccagatcacaatgggcatgccctatgcc

SEQ ID NO: 139 - DNA, 51 bp, synthetic construct
  source 1..51: mol_type = other DNA; note = primer iTK3-2-94-Rv
acccgccgcactgcaggtaccgcaccgtgttggcaagtagcccataaacgc

SEQ ID NO: 140 - DNA, 54 bp, synthetic construct
  source 1..54: mol_type = other DNA; note = primer iTK3-2-90-Fw
gcggcggtggtgatgacaagtgcccagatcacaatgggaatgccttacgccgtg

SEQ ID NO: 141 - DNA, 51 bp, synthetic construct
  source 1..51: mol_type = other DNA; note = primer iTK3-2-90-Rv
acccgccacactgcaggtaccgcacggtattggccagtagcccataaacgc

SEQ ID NO: 142 - DNA, 41 bp, synthetic construct
  source 1..41: mol_type = other DNA; note = primer iTK3-3-98-Fw
cagcgccccggcgagcggctggacctggctatgctcgctgc

SEQ ID NO: 143 - DNA, 31 bp, synthetic construct
  source 1..31: mol_type = other DNA; note = primer iTK3-3-98-Rv
gggcgtcccggcagccggcgggcgactggtc

SEQ ID NO: 144 - DNA, 50 bp, synthetic construct
  source 1..50: mol_type = other DNA; note = primer iTK3-3-94-Fw
cagcgccccggcgagcgcctggacctggccatgctggctgcgatccgccg

SEQ ID NO: 145 - DNA, 44 bp, synthetic construct
  source 1..44: mol_type = other DNA; note = primer iTK3-3-94-Rv
gggcgtcccggcatccggcgggcgactggtcgtaatcgaggata

SEQ ID NO: 146 - DNA, 53 bp, synthetic construct
  source 1..53: mol_type = other DNA; note = primer iTK3-3-90-Fw
cagcgccccggagagcggctcgacctggccatgctggccgcgattcggcgcgt

SEQ ID NO: 147 - DNA, 49 bp, synthetic construct
  source 1..49: mol_type = other DNA; note = primer iTK3-3-90-Rv
gggcgtcgcggcagccagcgggcgactggtcgtagtccaggatgaagac

SEQ ID NO: 148 - DNA, 330 bp, synthetic construct
  source 1..330: mol_type = other DNA; note = SceTK3 gene
  CDS 1..141: protein_id = 149; translation = MASYPGHQHASAFDQAARSRGHSNRRTALRPRRQQEATEVRPEQKK
  CDS 142..162: protein_id = 150; translation = RVGITG
  CDS 163..330: protein_id = 151; translation = CIVFILDYDQSPAGCRDALLQLTSGMVQTHVTTPGSIPTICDLARTFAREMGEAN
atggcttcgtaccccggccatcaacacgcgtctgcgttcgaccaggctgcgcgttctcgcggccatagcaaccgacgtacggcgttgcgccctcgccggcagcaagaagccacggaagtccgcccggagcagaaaaagtgacgcgtagggataacagggtaatgcatcgtctttatcctggattacgaccaatcgcccgccggctgccgggacgccctgctgcaacttacctccgggatggtccagacccacgtcaccacccccggctccataccgacgatatgcgacctggcgcgcacgtttgcccgggagatgggggaggctaactga

SEQ ID NO: 149 - protein, 46 aa, synthetic construct
MASYPGHQHASAFDQAARSRGHSNRRTALRPRRQQEATEVRPEQKK

SEQ ID NO: 150 - protein, 6 aa, synthetic construct
RVGITG

SEQ ID NO: 151 - protein, 55 aa, synthetic construct
CIVFILDYDQSPAGCRDALLQLTSGMVQTHVTTPGSIPTICDLARTFAREMGEAN

SEQ ID NO: 152 - DNA, 362 bp, synthetic construct
  source 1..362: mol_type = other DNA; note = iTK3-1-100 gene
gcgccctcgccggcagcaagaagccacggaagtccgcccggagcagaaaatgcccacgctactgcgggtttatatagacggtccccacgggatggggaaaaccaccaccacgcaactgctggtggccctgggttcgcgcgacgatatcgtctacgtacccgagccgatgacttactggcgggtgctgggggcttccgagacaatcgcgaacatctacaccacacaacaccgcctcgaccagggtgagatatcggccggggacgcggcggtggtaatgacaagcgcccagataacaatgggcatgccttatgccgtgaccgacgccgttctggctcctcatatcgggggggaggctgggagct

SEQ ID NO: 153 - DNA, 412 bp, synthetic construct
  source 1..412: mol_type = other DNA; note = iTK3-2-100 gene
gcggcggtggtaatgacaagcgcccagataacaatgggcatgccttatgccgtgaccgacgccgttctggctcctcatatcgggggggaggctgggagctcacatgccccgcccccggccctcaccctcatcttcgaccgccatcccatcgccgccctcctgtgctacccggccgcgcggtaccttatgggcagcatgaccccccaggccgtgctggcgttcgtggccctcatcccgccgaccttgcccggcaccaacatcgtgcttggggcccttccggaggacagacacatcgaccgcctggccaaacgccagcgccccggcgagcggctggacctggctatgctggctgcgattcgccgcgtttacgggctacttgccaatacggtgcggtatctgcagtgcggcgggt

SEQ ID NO: 154 - DNA, 358 bp, synthetic construct
  source 1..358: mol_type = other DNA; note = iTK3-3-100 gene
cagcgccccggcgagcggctggacctggctatgctggctgcgattcgccgcgtttacgggctacttgccaatacggtgcggtatctgcagtgcggcgggtcgtggcgggaggactggggacagctttcggggacggccgtgccgccccagggtgccgagccccagagcaacgcgggcccacgaccccatatcggggacacgttatttaccctgtttcgggcccccgagttgctggcccccaacggcgacctgtataacgtgtttgcctgggccttggacgtcttggccaaacgcctccgttccatgcacgtctttatcctggattacgaccaatcgcccgccggctgccgggacgccc

SEQ ID NO: 155 - DNA, 362 bp, synthetic construct
  source 1..362: mol_type = other DNA; note = iTK3-1-98 gene
gcgccctcgccggcagcaagaagctacggaagtccgcccggagcagaaaatgcccacgctactgcgggtttatatagacggtccccacgggatggggaaaaccaccaccacgcaactgctggtggccctgggttcgcgcgacgatatcgtctacgtacccgagccgatgacttactggcgggtgctgggggcttccgagacaatcgcgaacatctacaccacacaacaccgcctcgaccagggtgagatatcggccggggacgcggcggtggtaatgacaagcgcccagataacaatgggcatgccttatgccgtgaccgacgccgtgctggctcctcatatcgggggggaggctgggagct

SEQ ID NO: 156 - DNA, 362 bp, synthetic construct
  source 1..362: mol_type = other DNA; note = iTK3-1-94 gene
gcgccctcgccgccagcaagaagctacggaagtccggccggagcagaaaatgcccacgctactgcgggtttatatagacggtccccacgggatggggaaaaccaccaccacgcaactgctggtggccctgggttcgcgcgacgatatcgtctacgtacccgagccgatgacttactggcgggtgctgggggcttccgagacaatcgcgaacatctacaccacacaacaccgcctcgaccagggtgagatatcggccggggacgcggcggtggtaatgacaagcgcccagataacaatgggcatgccttatgccgtgacagacgccgttctggcccctcatatcggcggggaggctgggagct

SEQ ID NO: 157 - DNA, 362 bp, synthetic construct
  source 1..362: mol_type = other DNA; note = iTK3-1-90 gene
gcgcccccgccggcaacaagaagctacggaagtgcgcccggaacagaaaatgcccacgctactgcgggtttatatagacggtccccacgggatggggaaaaccaccaccacgcaactgctggtggccctgggttcgcgcgacgatatcgtctacgtacccgagccgatgacttactggcgggtgctgggggcttccgagacaatcgcgaacatctacaccacacaacaccgcctcgaccagggtgagatatcggccggggacgcggcggtggtaatgacaagcgcccagataacaatgggcatgccttatgccgtgacagacgccgtgctggctccccatatcggcggggaggccgggagct

SEQ ID NO: 158 - DNA, 412 bp, synthetic construct
  source 1..412: mol_type = other DNA; note = iTK3-2-98 gene
gcggcggtggtaatgacaagcgcccagataaccatgggcatgccttatgccgtgaccgacgccgttctggctcctcatatcgggggggaggctgggagctcacatgccccgcccccggccctcaccctcatcttcgaccgccatcccatcgccgccctcctgtgctacccggccgcgcggtaccttatgggcagcatgaccccccaggccgtgctggcgttcgtggccctcatcccgccgaccttgcccggcaccaacatcgtgcttggggcccttccggaggacagacacatcgaccgcctggccaaacgccagcgccccggcgagcggctggacctggctatgctggctgcgattcgccgcgtttacgggctacttgctaatacggtgcggtatctgcagtgcggcgggt

SEQ ID NO: 159 - DNA, 412 bp, synthetic construct
  source 1..412: mol_type = other DNA; note = iTK3-2-94 gene
gcggcggtggtaatgaccagcgcccagatcacaatgggcatgccctatgccgtgaccgacgccgttctggctcctcatatcgggggggaggctgggagctcacatgccccgcccccggccctcaccctcatcttcgaccgccatcccatcgccgccctcctgtgctacccggccgcgcggtaccttatgggcagcatgaccccccaggccgtgctggcgttcgtggccctcatcccgccgaccttgcccggcaccaacatcgtgcttggggcccttccggaggacagacacatcgaccgcctggccaaacgccagcgccccggcgagcggctggacctggctatgctggctgcgattcgccgcgtttatgggctacttgccaacacggtgcggtacctgcagtgcggcgggt

SEQ ID NO: 160 - DNA, 412 bp, synthetic construct
  source 1..412: mol_type = other DNA; note = iTK3-2-90 gene
gcggcggtggtgatgacaagtgcccagatcacaatgggaatgccttacgccgtgaccgacgccgttctggctcctcatatcgggggggaggctgggagctcacatgccccgcccccggccctcaccctcatcttcgaccgccatcccatcgccgccctcctgtgctacccggccgcgcggtaccttatgggcagcatgaccccccaggccgtgctggcgttcgtggccctcatcccgccgaccttgcccggcaccaacatcgtgcttggggcccttccggaggacagacacatcgaccgcctggccaaacgccagcgccccggcgagcggctggacctggctatgctggctgcgattcgccgcgtttatgggctactggccaataccgtgcggtacctgcagtgtggcgggt

SEQ ID NO: 161 - DNA, 358 bp, synthetic construct
  source 1..358: mol_type = other DNA; note = iTK3-3-98 gene
cagcgccccggcgagcggctggacctggctatgctcgctgcgattcgccgcgtttacgggctacttgccaatacggtgcggtatctgcagtgcggcgggtcgtggcgggaggactggggacagctttcggggacggccgtgccgccccagggtgccgagccccagagcaacgcgggcccacgaccccatatcggggacacgttatttaccctgtttcgggcccccgagttgctggcccccaacggcgacctgtataacgtgtttgcctgggccttggacgtcttggccaaacgcctccgttccatgcacgtctttatcctggattacgaccagtcgcccgccggctgccgggacgccc

SEQ ID NO: 162 - DNA, 358 bp, synthetic construct
  source 1..358: mol_type = other DNA; note = iTK3-3-94 gene
cagcgccccggcgagcgcctggacctggccatgctggctgcgatccgccgcgtttacgggctacttgccaatacggtgcggtatctgcagtgcggcgggtcgtggcgggaggactggggacagctttcggggacggccgtgccgccccagggtgccgagccccagagcaacgcgggcccacgaccccatatcggggacacgttatttaccctgtttcgggcccccgagttgctggcccccaacggcgacctgtataacgtgtttgcctgggccttggacgtcttggccaaacgcctccgttccatgcacgtctttatcctcgattacgaccagtcgcccgccggatgccgggacgccc

SEQ ID NO: 163 - DNA, 358 bp, synthetic construct
  source 1..358: mol_type = other DNA; note = iTK3-3-90 gene
cagcgccccggagagcggctcgacctggccatgctggccgcgattcggcgcgtttacgggctacttgccaatacggtgcggtatctgcagtgcggcgggtcgtggcgggaggactggggacagctttcggggacggccgtgccgccccagggtgccgagccccagagcaacgcgggcccacgaccccatatcggggacacgttatttaccctgtttcgggcccccgagttgctggcccccaacggcgacctgtataacgtgtttgcctgggccttggacgtcttggccaaacgcctccgttccatgcacgtcttcatcctggactacgaccagtcgcccgctggctgccgcgacgccc

SEQ ID NO: 164 - DNA, 57 bp, synthetic construct
  source 1..57: mol_type = other DNA; note = nucleotide sequence encoding P2A
  CDS 1..57: protein_id = 165; translation = ATNFSLLKQAGDVEENPGP
gctactaacttcagcctgctgaagcaggctggagacgtggaggagaaccctggacct

SEQ ID NO: 165 - protein, 19 aa, synthetic construct
ATNFSLLKQAGDVEENPGP

SEQ ID NO: 166 - DNA, 60 bp, synthetic construct
  source 1..60: mol_type = other DNA; note = nucleotide sequence encoding E2A
  CDS 1..60: protein_id = 167; translation = QCTNYALLKLAGDVESNPGP
caatgtactaactacgctttgttgaaactcgctggcgatgttgaaagtaaccccggtcct

SEQ ID NO: 167 - protein, 20 aa, synthetic construct
QCTNYALLKLAGDVESNPGP

SEQ ID NO: 168 - DNA, 66 bp, synthetic construct
  source 1..66: mol_type = other DNA; note = nucleotide sequence encoding F2A
  CDS 1..66: protein_id = 169; translation = VKQTLNFDLLKLAGDVESNPGP
gtgaaacagactttgaattttgaccttctcaagttggcgggagacgtggagtccaacccagggccc

SEQ ID NO: 169 - protein, 22 aa, synthetic construct
VKQTLNFDLLKLAGDVESNPGP

SEQ ID NO: 170 - DNA, 596 bp, synthetic construct
  source 1..596: mol_type = other DNA; note = IRES sequence
aattccgcccctctcccccccccccctctccctcccccccccctaacgttactggccgaagccgcttggaataaggccggtgtgcgtttgtctatatgtgattttccaccatattgccgtcttttggcaatgtgagggcccggaaacctggccctgtcttcttgacgagcattcctaggggtctttcccctctcgccaaaggaatgcaaggtctgttgaatgtcgtgaaggaagcagttcctctggaagcttcttgaagacaaacaacgtctgtagcgaccctttgcaggcagcggaaccccccacctggcgacaggtgcctctgcggccaaaagccacgtgtataagatacacctgcaaaggcggcacaaccccagtgccacgttgtgagttggatagttgtggaaagagtcaaatggctctcctcaagcgtattcaacaaggggctgaaggatgcccagaaggtaccccattgtatgggatctgatctggggcctcggtgcacatgctttacatgtgtttagtcgaggttaaaaaaacgtctaggccccccgaaccacggggacgtggttttcctttgaaaaacacgatgataa

SEQ ID NO: 171 - DNA, 585 bp, synthetic construct
  source 1..585: mol_type = other DNA; note = IRES2 sequence
gcccctctccctcccccccccctaacgttactggccgaagccgcttggaataaggccggtgtgcgtttgtctatatgttattttccaccatattgccgtcttttggcaatgtgagggcccggaaacctggccctgtcttcttgacgagcattcctaggggtctttcccctctcgccaaaggaatgcaaggtctgttgaatgtcgtgaaggaagcagttcctctggaagcttcttgaagacaaacaacgtctgtagcgaccctttgcaggcagcggaaccccccacctggcgacaggtgcctctgcggccaaaagccacgtgtataagatacacctgcaaaggcggcacaaccccagtgccacgttgtgagttggatagttgtggaaagagtcaaatggctctcctcaagcgtattcaacaaggggctgaaggatgcccagaaggtaccccattgtatgggatctgatctggggcctcggtacacatgctttacatgtgtttagtcgaggttaaaaaaacgtctaggccccccgaaccacggggacgtggttttcctttgaaaaacacgatgataatatggccaca

SEQ ID NO: 172 - DNA, 711 bp, synthetic construct
  source 1..711: mol_type = other DNA; note = mNeonGreen gene
  CDS 1..711: protein_id = 173; translation = MVSKGEEDNMASLPATHELHIFGSINGVDFDMVGQGTGNPNDGYEELNLKSTKGDLQFSPWILVPHIGYGFHQYLPYPDGMSPFQAAMVDGSGYQVHRTMQFEDGASLTVNYRYTYEGSHIKGEAQVKGTGFPADGPVMTNSLTAADWCRSKKTYPNDKTIISTFKWSYTTGNGKRYRSTARTTYTFAKPMAANYLKNQPMYVFRKTELKHSKTELNFKEWQKAFTDVMGMDELYK
atggtgtccaagggcgaagaggacaacatggccagcctgcctgccacccacgagctgcacatcttcggcagcatcaacggcgtggacttcgacatggtgggacagggcaccggcaaccccaacgacggctacgaggaactgaacctgaagtccacaaagggcgacctgcagttcagcccctggattctggtgccccacatcggctacggcttccaccagtacctgccctaccccgacggcatgagccctttccaggccgctatggtggatggcagcggctaccaggtgcaccggaccatgcagtttgaggacggcgccagcctgaccgtgaactaccggtacacatacgagggcagccacatcaagggcgaggcccaagtgaagggcacaggctttccagccgacggccccgtgatgaccaatagcctgacagccgccgactggtgcagaagcaagaaaacctaccccaatgacaagaccatcatcagcaccttcaagtggtcctacaccaccggcaatggcaagcggtacagaagcaccgcccggaccacctacaccttcgccaaacctatggccgccaactacctgaagaaccagcctatgtacgtgttccgcaagaccgagctgaagcactccaagacagaactgaacttcaaagagtggcagaaagccttcaccgacgtgatgggcatggacgagctgtacaagtga

SEQ ID NO: 173 - protein, 236 aa, synthetic construct
MVSKGEEDNMASLPATHELHIFGSINGVDFDMVGQGTGNPNDGYEELNLKSTKGDLQFSPWILVPHIGYGFHQYLPYPDGMSPFQAAMVDGSGYQVHRTMQFEDGASLTVNYRYTYEGSHIKGEAQVKGTGFPADGPVMTNSLTAADWCRSKKTYPNDKTIISTFKWSYTTGNGKRYRSTARTTYTFAKPMAANYLKNQPMYVFRKTELKHSKTELNFKEWQKAFTDVMGMDELYK

SEQ ID NO: 174 - DNA, 1185 bp, synthetic construct
  source 1..1185: mol_type = other DNA; note = GeNL gene
  CDS 1..1185: protein_id = 175; translation = MVSKGEEDNMASLPATHELHIFGSINGVDFDMVGQGTGNPNDGYEELNLKSTKGDLQFSPWILVPHIGYGFHQYLPYPDGMSPFQAAMVDGSGYQVHRTMQFEDGASLTVNYRYTYEGSHIKGEAQVKGTGFPADGPVMTNSLTAADWCRSKKTYPNDKTIISTFKWSYTTGNGKRYRSTARTTYTFAKPMAANYLKNQPMYVFRKTELKHSKTELNFKEWQKAFTGFEDFVGDWRQTAGYNLDQVLEQGGVSSLFQNLGVSVTPIQRIVLSGENGLKIDIHVIIPYEGLSGDQMGQIEKIFKVVYPVDDHHFKVILHYGTLVIDGVTPNMIDYFGRPYEGIAVFDGKKITVTGTLWNGNKIIDERLINPDGSLLFRVTINGVTGWRLCERILA
atggtgtccaagggcgaagaggacaacatggccagcctgcctgccacccacgagctgcacatcttcggcagcatcaacggcgtggacttcgacatggtgggacagggcaccggcaaccccaacgacggctacgaggaactgaacctgaagtccacaaagggcgacctgcagttcagcccctggattctggtgccccacatcggctacggcttccaccagtacctgccctaccccgacggcatgagccctttccaggccgctatggtggatggcagcggctaccaggtgcaccggaccatgcagtttgaggacggcgccagcctgaccgtgaactaccggtacacatacgagggcagccacatcaagggcgaggcccaagtgaagggcacaggctttccagccgacggccccgtgatgaccaatagcctgacagccgccgactggtgcagaagcaagaaaacctaccccaatgacaagaccatcatcagcaccttcaagtggtcctacaccaccggcaatggcaagcggtacagaagcaccgcccggaccacctacaccttcgccaaacctatggccgccaactacctgaagaaccagcctatgtacgtgttccgcaagaccgagctgaagcactccaagacagaactgaacttcaaagagtggcagaaagccttcaccgggtttgaagatttcgttggggactggcgacagacagccggctacaacctggaccaagtccttgaacagggaggtgtgtccagtttgtttcagaatctcggggtgtccgtaactccgatccaaaggattgtcctgagcggtgaaaatgggctgaagatcgacatccatgtcatcatcccgtatgaaggtctgagcggcgaccaaatgggccagatcgaaaaaatttttaaggtggtgtaccctgtggatgatcatcactttaaggtgatcctgcactatggcacactggtaatcgacggggttacgccgaacatgatcgactatttcggacggccgtatgaaggcatcgccgtgttcgacggcaaaaagatcactgtaacagggaccctgtggaacggcaacaaaattatcgacgagcgcctgatcaaccccgacggctccctgctgttccgagtaaccatcaacggagtgaccggctggcggctgtgcgaacgcattctggcgtaa

SEQ ID NO: 175 - protein, 394 aa, synthetic construct
MVSKGEEDNMASLPATHELHIFGSINGVDFDMVGQGTGNPNDGYEELNLKSTKGDLQFSPWILVPHIGYGFHQYLPYPDGMSPFQAAMVDGSGYQVHRTMQFEDGASLTVNYRYTYEGSHIKGEAQVKGTGFPADGPVMTNSLTAADWCRSKKTYPNDKTIISTFKWSYTTGNGKRYRSTARTTYTFAKPMAANYLKNQPMYVFRKTELKHSKTELNFKEWQKAFTGFEDFVGDWRQTAGYNLDQVLEQGGVSSLFQNLGVSVTPIQRIVLSGENGLKIDIHVIIPYEGLSGDQMGQIEKIFKVVYPVDDHHFKVILHYGTLVIDGVTPNMIDYFGRPYEGIAVFDGKKITVTGTLWNGNKIIDERLINPDGSLLFRVTINGVTGWRLCERILA

SEQ ID NO: 176 - DNA, 1185 bp, synthetic construct
  source 1..1185: mol_type = other DNA; note = SceGeNL gene
  CDS 1..894: protein_id = 177; translation = MVSKGEEDNMASLPATHELHIFGSINGVDFDMVGQGTGNPNDGYEELNLKSTKGDLQFSPWILVPHIGYGFHQYLPYPDGMSPFQAAMVDGSGYQVHRTMQFEDGASLTVNYRYTYEGSHIKGEAQVKGTGFPADGPVMTNSLTAADWCRSKKTYPNDKTIISTFKWSYTTGNGKRYRSTARTTYTFAKPMAANYLKNQPMYVFRKTELKHSKTELNFKEWQKAFTGFEDFVGDWRQTAGYNLDQVLEQGGVSSLFQNLGVSVTPIQRIVLSGENGLKIDIHVIIPYEGLSGDQMGQ
  CDS 904..1185: protein_id = 178; translation = QGNVYPVDDHHFKVILHYGTLVIDGVTPNMIDYFGRPYEGIAVFDGKKITVTGTLWNGNKIIDERLINPDGSLLFRVTINGVTGWRLCERILA
atggtgtccaagggcgaagaggacaacatggccagcctgcctgccacccacgagctgcacatcttcggcagcatcaacggcgtggacttcgacatggtgggacagggcaccggcaaccccaacgacggctacgaggaactgaacctgaagtccacaaagggcgacctgcagttcagcccctggattctggtgccccacatcggctacggcttccaccagtacctgccctaccccgacggcatgagccctttccaggccgctatggtggatggcagcggctaccaggtgcaccggaccatgcagtttgaggacggcgccagcctgaccgtgaactaccggtacacatacgagggcagccacatcaagggcgaggcccaagtgaagggcacaggctttccagccgacggccccgtgatgaccaatagcctgacagccgccgactggtgcagaagcaagaaaacctaccccaatgacaagaccatcatcagcaccttcaagtggtcctacaccaccggcaatggcaagcggtacagaagcaccgcccggaccacctacaccttcgccaaacctatggccgccaactacctgaagaaccagcctatgtacgtgttccgcaagaccgagctgaagcactccaagacagaactgaacttcaaagagtggcagaaagccttcaccgggtttgaagatttcgttggggactggcgacagacagccggctacaacctggaccaagtccttgaacagggaggtgtgtccagtttgtttcagaatctcggggtgtccgtaactccgatccaaaggattgtcctgagcggtgaaaatgggctgaagatcgacatccatgtcatcatcccgtatgaaggtctgagcggcgaccaaatgggccagtgatagggataacagggtaatgtgtaccctgtggatgatcatcactttaaggtgatcctgcactatggcacactggtaatcgacggggttacgccgaacatgatcgactatttcggacggccgtatgaaggcatcgccgtgttcgacggcaaaaagatcactgtaacagggaccctgtggaacggcaacaaaattatcgacgagcgcctgatcaaccccgacggctccctgctgttccgagtaaccatcaacggagtgaccggctggcggctgtgcgaacgcattctggcgtaa

SEQ ID NO: 177 - protein, 297 aa, synthetic construct
MVSKGEEDNMASLPATHELHIFGSINGVDFDMVGQGTGNPNDGYEELNLKSTKGDLQFSPWILVPHIGYGFHQYLPYPDGMSPFQAAMVDGSGYQVHRTMQFEDGASLTVNYRYTYEGSHIKGEAQVKGTGFPADGPVMTNSLTAADWCRSKKTYPNDKTIISTFKWSYTTGNGKRYRSTARTTYTFAKPMAANYLKNQPMYVFRKTELKHSKTELNFKEWQKAFTGFEDFVGDWRQTAGYNLDQVLEQGGVSSLFQNLGVSVTPIQRIVLSGENGLKIDIHVIIPYEGLSGDQMGQ

SEQ ID NO: 178 - protein, 93 aa, synthetic construct; identical to SEQ ID NO: 11

SEQ ID NO: 179 - DNA, 1131 bp, synthetic construct
  source 1..1131: mol_type = other DNA; note = TK30 gene
  CDS 1..1131: protein_id = 180; translation = MASYPGHQHASAFDQAARSRGHSNRRTALRPRRQQEATEVRPEQKMPTLLRVYIDGPHGMGKTTTTQLLVALGSRDDIVYVPEPMTYWRVLGASETIANIYTTQHRLDQGEISAGDAAVVMTSAQITMGMPYAVTDAVLAPHIGGEAGSSHVPPPALTILADRHPIAYFLCYPAARYLMGSMTPQAVLAFVALIPPTLPGTNIVLGALPEDRHIDRLAKRQRPGERLDLAMLAAIRRVYGLLANTVRYLQCGGSWREDWGQLSGTAVPPQGAEPQSNAGPRPHIGDTLFTLFRAPELLAPNGDLYNVFAWALDVLAKRLRSMHVFILDYDQSPAGCRDALLQLTSGMVQTHVTTPGSIPTICDLARTFAREMGEAN
atggcttcgtaccccggccatcaacacgcgtctgcgttcgaccaggctgcgcgttctcgcggccatagcaaccgacgtacggcgttgcgccctcgccggcagcaagaagccacggaagtccgcccggagcagaaaatgcccacgctactgcgggtttatatagacggtccccacgggatggggaaaaccaccaccacgcaactgctggtggccctgggttcgcgcgacgatatcgtctacgtacccgagccgatgacttactggcgggtgctgggggcttccgagacaatcgcgaacatctacaccacacaacaccgcctcgaccagggtgagatatcggccggggacgcggcggtggtaatgacaagcgcccagataacaatgggcatgccttatgccgtgaccgacgccgttctggctcctcatatcgggggggaggctgggagctcacatgtgccgcccccggccctcaccatcctggccgaccgccatcccatcgcctacttcctgtgctacccggccgcgcggtaccttatgggcagcatgaccccccaggccgtgctggcgttcgtggccctcatcccgccgaccttgcccggcaccaacatcgtgcttggggcccttccggaggacagacacatcgaccgcctggccaaacgccagcgccccggcgagcggctggacctggctatgctggctgcgattcgccgcgtttacgggctacttgccaatacggtgcggtatctgcagtgcggcgggtcgtggcgggaggactggggacagctttcggggacggccgtgccgccccagggtgccgagccccagagcaacgcgggcccacgaccccatatcggggacacgttatttaccctgtttcgggcccccgagttgctggcccccaacggcgacctgtataacgtgtttgcctgggccttggacgtcttggccaaacgcctccgttccatgcacgtctttatcctggattacgaccaatcgcccgccggctgccgggacgccctgctgcaacttacctccgggatggtccagacccacgtcaccacccccggctccataccgacgatatgcgacctggcgcgcacgtttgcccgggagatgggggaggctaactga

SEQ ID NO: 180 - protein, 376 aa, synthetic construct
MASYPGHQHASAFDQAARSRGHSNRRTALRPRRQQEATEVRPEQKMPTLLRVYIDGPHGMGKTTTTQLLVALGSRDDIVYVPEPMTYWRVLGASETIANIYTTQHRLDQGEISAGDAAVVMTSAQITMGMPYAVTDAVLAPHIGGEAGSSHVPPPALTILADRHPIAYFLCYPAARYLMGSMTPQAVLAFVALIPPTLPGTNIVLGALPEDRHIDRLAKRQRPGERLDLAMLAAIRRVYGLLANTVRYLQCGGSWREDWGQLSGTAVPPQGAEPQSNAGPRPHIGDTLFTLFRAPELLAPNGDLYNVFAWALDVLAKRLRSMHVFILDYDQSPAGCRDALLQLTSGMVQTHVTTPGSIPTICDLARTFAREMGEAN

SEQ ID NO: 181 - DNA, 412 bp, synthetic construct
  source 1..412: mol_type = other DNA; note = iTK303-2-100 gene
gcggcggtggtaatgacaagcgcccagataacaatgggcatgccttatgccgtgaccgacgccgttctggctcctcatatcgggggggaggctgggagctcacatgccccgcccccggccctcaccatcctggccgaccgccatcccatcgcctacttcctgtgctacccggccgcgcggtaccttatgggcagcatgaccccccaggccgtgctggcgttcgtggccctcatcccgccgaccttgcccggcaccaacatcgtgcttggggcccttccggaggacagacacatcgaccgcctggccaaacgccagcgccccggcgagcggctggacctggctatgctggctgcgattcgccgcgtttacgggctacttgccaatacggtgcggtatctgcagtgcggcgggt

SEQ ID NO: 182 - DNA, 412 bp, synthetic construct
  source 1..412: mol_type = other DNA; note = iTK303-2-98 gene
gcggcggtggtaatgacaagcgcccagataaccatgggcatgccttatgccgtgaccgacgccgttctggctcctcatatcgggggggaggctgggagctcacatgccccgcccccggccctcaccatcctggccgaccgccatcccatcgcctacttcctgtgctacccggccgcgcggtaccttatgggcagcatgaccccccaggccgtgctggcgttcgtggccctcatcccgccgaccttgcccggcaccaacatcgtgcttggggcccttccggaggacagacacatcgaccgcctggccaaacgccagcgccccggcgagcggctggacctggctatgctggctgcgattcgccgcgtttacgggctacttgctaatacggtgcggtatctgcagtgcggcgggt

SEQ ID NO: 183 - DNA, 412 bp, synthetic construct
  source 1..412: mol_type = other DNA; note = iTK303-2-94 gene
gcggcggtggtaatgaccagcgcccagatcacaatgggcatgccctatgccgtgaccgacgccgttctggctcctcatatcgggggggaggctgggagctcacatgccccgcccccggccctcaccatcctggccgaccgccatcccatcgcctacttcctgtgctacccggccgcgcggtaccttatgggcagcatgaccccccaggccgtgctggcgttcgtggccctcatcccgccgaccttgcccggcaccaacatcgtgcttggggcccttccggaggacagacacatcgaccgcctggccaaacgccagcgccccggcgagcggctggacctggctatgctggctgcgattcgccgcgtttatgggctacttgccaacacggtgcggtacctgcagtgcggcgggt

SEQ ID NO: 184 - DNA, 412 bp, synthetic construct
  source 1..412: mol_type = other DNA; note = iTK303-2-90 gene
gcggcggtggtgatgacaagtgcccagatcacaatgggaatgccttacgccgtgaccgacgccgttctggctcctcatatcgggggggaggctgggagctcacatgccccgcccccggccctcaccatcctggccgaccgccatcccatcgcctacttcctgtgctacccggccgcgcggtaccttatgggcagcatgaccccccaggccgtgctggcgttcgtggccctcatcccgccgaccttgcccggcaccaacatcgtgcttggggcccttccggaggacagacacatcgaccgcctggccaaacgccagcgccccggcgagcggctggacctggctatgctggctgcgattcgccgcgtttatgggctactggccaataccgtgcggtacctgcagtgtggcgggt

SEQ ID NO: 185 - DNA, 1122 bp, synthetic construct
  source 1..1122: mol_type = other DNA; note = CD::UPRT gene
  CDS 1..1122: protein_id = 186; translation = MVTGGMASKWDQKGMDIAYEEAALGYKEGGVPIGGCLINNKDGSVLGRGHNMRFQKGSATLHGEISTLENCGRLEGKVYKDTTLYTTLSPCDMCTGAIIMYGIPRCVVGENVNFKSKGEKYLQTRGHEVVVVDDERCKKIMKQFIDERPQDWFEDIGEASEPFKNVYLLPQTNQLLGLYTIIRNKNTTRPDFIFYSDRIIRLLVEEGLNHLPVQKQIVETDTNENFEGVSFMGKICGVSIVRAGESMEQGLRDCCRSVRIGKILIQRDEETALPKLFYEKLPEDISERYVFLLDPMLATGGSAIMATEVLIKRGVKPERIYFLNLICSKEGIEKYHAAFPEVRIVTGALDRGLDENKYLVPGLGDFGDRYYCV
atggtcacaggaggcatggcttcaaagtgggaccagaagggcatggacattgcctatgaggaggctgctctgggctacaaggagggaggggtcccaattggtggctgcctcatcaacaacaaggatggcagtgtcctgggcaggggccacaacatgaggttccagaagggcagtgccaccctgcatggggagatcagcaccctggagaactgtggcaggctggagggcaaggtctacaaggacaccactctgtacaccaccctcagcccttgtgacatgtgcacaggggccatcatcatgtatggcattcccaggtgtgtggtgggagagaatgtcaacttcaagtcaaaaggagagaagtacctccagaccaggggccatgaggtggttgtggtggatgatgagaggtgcaagaagattatgaagcagttcattgatgagagaccccaggactggtttgaggacattggggaggcctctgagcccttcaagaatgtgtacctcctcccccagaccaaccaactcctgggactctacaccatcatcaggaacaagaacaccaccaggccagacttcatcttctacagtgacaggatcatcaggctcctggtggaggagggcctcaaccacctccctgtgcagaagcagattgtggagactgacaccaatgagaactttgagggagtgtctttcatgggcaagatttgtggggtgtccattgtgagggctggggagagcatggagcagggcctgagggactgttgcaggagtgtgaggattggcaagatcctgatccagagggatgaggagactgccctgcccaagctgttctatgagaagctccctgaagacatctctgagaggtatgtcttcctcctggaccccatgctggcaactggaggctctgcaatcatggccactgaggtgctcatcaagaggggagtcaagcctgagaggatctacttcctcaacctcatctgctcaaaggagggcattgagaagtaccatgctgccttccctgaagtgaggattgtcactggggctctggacaggggcctggatgagaacaagtacctggtccctggcctgggagactttggggacagatactactgtgtctaa

SEQ ID NO: 186 - protein, 373 aa, synthetic construct
MVTGGMASKWDQKGMDIAYEEAALGYKEGGVPIGGCLINNKDGSVLGRGHNMRFQKGSATLHGEISTLENCGRLEGKVYKDTTLYTTLSPCDMCTGAIIMYGIPRCVVGENVNFKSKGEKYLQTRGHEVVVVDDERCKKIMKQFIDERPQDWFEDIGEASEPFKNVYLLPQTNQLLGLYTIIRNKNTTRPDFIFYSDRIIRLLVEEGLNHLPVQKQIVETDTNENFEGVSFMGKICGVSIVRAGESMEQGLRDCCRSVRIGKILIQRDEETALPKLFYEKLPEDISERYVFLLDPMLATGGSAIMATEVLIKRGVKPERIYFLNLICSKEGIEKYHAAFPEVRIVTGALDRGLDENKYLVPGLGDFGDRYYCV

SEQ ID NO: 187 - DNA, 403 bp, synthetic construct
  source 1..403: mol_type = other DNA; note = SceCDUPRT3 gene
  CDS 1..168: protein_id = 188; translation = MVTGGMASKWDQKGMDIAYEEAALGYKEGGVPIGGCLINNKDGSVLGRGHNMRFQK
atggtcacaggaggcatggcttcaaagtgggaccagaagggcatggacattgcctatgaggaggctgctctgggctacaaggagggaggggtcccaattggtggctgcctcatcaacaacaaggatggcagtgtcctgggcaggggccacaacatgaggttccagaagtgacgcgtagggataacagggtaatgcatacactgaggtgctcatcaagaggggagtcaagcctgagaggatctacttcctcaacctcatctgctcaaaggagggcattgagaagtaccatgctgccttccctgaagtgaggattgtcactggggctctggacaggggcctggatgagaacaagtacctggtccctggcctgggagactttggggacagatactactgtgtctaa

SEQ ID NO: 188 - protein, 56 aa, synthetic construct
MVTGGMASKWDQKGMDIAYEEAALGYKEGGVPIGGCLINNKDGSVLGRGHNMRFQK

SEQ ID NO: 189 - DNA, 23 bp, synthetic construct
  source 1..23: mol_type = other DNA; note = primer Sce-5'CDUPRT-Fw
taatacgactcactataggctag

SEQ ID NO: 190 - DNA, 49 bp, synthetic construct
  source 1..49: mol_type = other DNA; note = primer Sce-5'CDUPRT3-Rv
gcattaccctgttatccctacgcgtcacttctggaacctcatgttgtgg

SEQ ID NO: 191 - DNA, 46 bp, synthetic construct
  source 1..46: mol_type = other DNA; note = primer Sce-3'CDUPRT3-Fw
gtagggataacagggtaatgcatacactgaggtgctcatcaagagg

SEQ ID NO: 192 - DNA, 20 bp, synthetic construct
  source 1..20: mol_type = other DNA; note = primer Sce-3'CDUPRT-Rv
gagtgcaccatacgcggatc

SEQ ID NO: 193 - DNA, 20 bp, synthetic construct
  source 1..20: mol_type = other DNA; note = primer iCDUPRT3-1-100-Fw
acaaggatggcagtgtcctg

SEQ ID NO: 194 - DNA, 20 bp, synthetic construct
  source 1..20: mol_type = other DNA; note = primer iCDUPRT3-1-100-Rv
ctggtctggaggtacttctc

SEQ ID NO: 195 - DNA, 20 bp, synthetic construct
  source 1..20: mol_type = other DNA; note = primer iCDUPRT3-2-100-Fw
acatgtgcacaggggccatc

SEQ ID NO: 196 - DNA, 20 bp, synthetic construct
  source 1..20: mol_type = other DNA; note = primer iCDUPRT3-2-100-Rv
tctcattggtgtcagtctcc

SEQ ID NO: 197 - DNA, 21 bp, synthetic construct
  source 1..21: mol_type = other DNA; note = primer iCDUPRT3-3-100-Fw
ttcatcttctacagtgacagg

SEQ ID NO: 198 - DNA, 19 bp, synthetic construct
  source 1..19: mol_type = other DNA; note = primer iCDUPRT3-3-100-Rv
ggaagtagatcctctcagg

SEQ ID NO: 199 - DNA, 32 bp, synthetic construct
  source 1..32: mol_type = other DNA; note = primer iCDUPRT3-1-98-Fw
acaaggatggcagtgtcctgggcagaggccac

SEQ ID NO: 200 - DNA, 45 bp, synthetic construct
  source 1..45: mol_type = other DNA; note = primer iCDUPRT3-1-98-Rv
ctggtctggaggtacttctctccttttgacttgaaattgacattc

SEQ ID NO: 201 - DNA, 47 bp, synthetic construct
  source 1..47: mol_type = other DNA; note = primer iCDUPRT3-1-94-Fw
acaaggatgggagtgtcctgggcagaggccacaacatgagattccag

SEQ ID NO: 202 - DNA, 51 bp, synthetic construct
  source 1..51: mol_type = other DNA; note = primer iCDUPRT3-1-94-Rv
ctggtctggaggtatttctctccttttgatttgaagttgacattttctccc

SEQ ID NO: 203 - DNA, 50 bp, synthetic construct
  source 1..50: mol_type = other DNA; note = primer iCDUPRT3-1-90-Fw
acaaggacggcagtgtgctgggcagaggccacaatatgaggtttcagaag

SEQ ID NO: 204 - DNA, 51 bp, synthetic construct
  source 1..51: mol_type = other DNA; note = primer iCDUPRT3-1-90-Rv
ctggtctgcaggtacttttctcctttagacttgaaattgacattttctccc

SEQ ID NO: 205 - DNA, 40 bp, synthetic construct
  source 1..40: mol_type = other DNA; note = primer iCDUPRT3-2-98-Fw
acatgtgcacaggggccatcatcatgtatgggattcccag

SEQ ID NO: 206 - DNA, 43 bp, synthetic construct
  source 1..43: mol_type = other DNA; note = primer iCDUPRT3-2-98-Rv
tctcattggtgtcagtctccacaatctgcttctggacagggag

SEQ ID NO: 207 - DNA, 51 bp, synthetic construct
  source 1..51: mol_type = other DNA; note = primer iCDUPRT3-2-94-Fw
acatgtgcacaggcgccatcatcatgtacggcattcccaggtgcgtggtgg

SEQ ID NO: 208 - DNA, 53 bp, synthetic construct
  source 1..53: mol_type = other DNA; note = primer iCDUPRT3-2-94-Rv
tctcattggtgtctgtctccacaatctgtttctgcacagggagatggttgagg

SEQ ID NO: 209 - DNA, 54 bp, synthetic construct
  source 1..54: mol_type = other DNA; note = primer iCDUPRT3-2-90-Fw
acatgtgcactggggccattatcatgtacggcattcctaggtgtgtcgtgggag

SEQ ID NO: 210 - DNA, 53 bp, synthetic construct
  source 1..53: mol_type = other DNA; note = primer iCDUPRT3-2-90-Rv
tctcattcgtgtcagtttccacaatttgcttctggacagggagatggttgagg

SEQ ID NO: 211 - DNA, 39 bp, synthetic construct
  source 1..39: mol_type = other DNA; note = primer iCDUPRT3-3-98-Fw
ttcatcttctacagtgacaggatcatcaggctgctggtg

SEQ ID NO: 212 - DNA, 32 bp, synthetic construct
  source 1..32: mol_type = other DNA; note = primer iCDUPRT3-3-98-Rv
ggaagtagatcctctcaggcttgacacccctc

SEQ ID NO: 213 - DNA, 51 bp, synthetic construct
  source 1..51: mol_type = other DNA; note = primer iCDUPRT3-3-94-Fw
ttcatcttctacagcgacaggatcatcagactcctggtggaggaaggcctc

SEQ ID NO: 214 - DNA, 44 bp, synthetic construct
  source 1..44: mol_type = other DNA; note = primer iCDUPRT3-3-94-Rv
ggaagtagatcctttcaggcttgacacccctcttgatcagcacc

SEQ ID NO: 215 - DNA, 55 bp, synthetic construct
  source 1..55: mol_type = other DNA; note = primer iCDUPRT3-3-90-Fw
ttcatcttctatagtgacagaatcatcagactcctggtcgaggaggggctcaacc

SEQ ID NO: 216 - DNA, 50 bp, synthetic construct
  source 1..50: mol_type = other DNA; note = primer iCDUPRT3-3-90-Rv
ggaagtaaatcctctctggcttgacacccctcttaatgagcacttcagtg

SEQ ID NO: 217 - DNA, 256 bp, synthetic construct
  source 1..256: mol_type = other DNA
acaaggatggcagtgtcctgggcaggggccacaacatgaggttccagaagggcagtgccaccctgcatggggagatcagcaccctggagaactgtggcaggctggagggcaaggtctacaaggacaccactctgtacaccaccctcagcccttgtgacatgtgcacaggggccatcatcatgtatggcattcccaggtgtgtggtgggagagaatgtcaacttcaagtcaaaaggagagaagtacctccagaccag

SEQ ID NO: 218 - DNA, 399 bp, synthetic construct
  source 1..399: mol_type = other DNA; note = iCDUPRT3-2-100 gene
acatgtgcacaggggccatcatcatgtatggcattcccaggtgtgtggtgggagagaatgtcaacttcaagtcaaaaggagagaagtacctccagaccaggggccatgaggtggttgtggtggatgatgagaggtgcaagaagattatgaagcagttcattgatgagagaccccaggactggtttgaggacattggggaggcctctgagcccttcaagaatgtgtacctcctcccccagaccaaccaactcctgggactctacaccatcatcaggaacaagaacaccaccaggccagacttcatcttctacagtgacaggatcatcaggctcctggtggaggagggcctcaaccacctccctgtgcagaagcagattgtggagactgacaccaatgaga

SEQ ID NO: 219 - DNA, 394 bp, synthetic construct
  source 1..394: mol_type = other DNA; note = iCDUPRT3-3-100 gene
ttcatcttctacagtgacaggatcatcaggctcctggtggaggagggcctcaaccacctccctgtgcagaagcagattgtggagactgacaccaatgagaactttgagggagtgtctttcatgggcaagatttgtggggtgtccattgtgagggctggggagagcatggagcagggcctgagggactgttgcaggagtgtgaggattggcaagatcctgatccagagggatgaggagactgccctgcccaagctgttctatgagaagctccctgaagacatctctgagaggtatgtcttcctcctggaccccatgctggcaactggaggctctgcaatcatggccactgaggtgctcatcaagaggggagtcaagcctgagaggatctacttcc

SEQ ID NO: 220 - DNA, 256 bp, synthetic construct
  source 1..256: mol_type = other DNA; note = iCDUPRT3-1-98 gene
acaaggatggcagtgtcctgggcagaggccacaacatgaggttccagaagggcagtgccaccctgcatggggagatcagcaccctggagaactgtggcaggctggagggcaaggtctacaaggacaccactctgtacaccaccctcagcccttgtgacatgtgcacaggggccatcatcatgtatggcattcccaggtgtgtggtgggagagaatgtcaatttcaagtcaaaaggagagaagtacctccagaccag

SEQ ID NO: 221 - DNA, 256 bp, synthetic construct
  source 1..256: mol_type = other DNA; note = iCDUPRT3-1-94 gene
acaaggatgggagtgtcctgggcagaggccacaacatgagattccagaagggcagtgccaccctgcatggggagatcagcaccctggagaactgtggcaggctggagggcaaggtctacaaggacaccactctgtacaccaccctcagcccttgtgacatgtgcacaggggccatcatcatgtatggcattcccaggtgtgtggtgggagaaaatgtcaacttcaaatcaaaaggagagaaatacctccagaccag

SEQ ID NO: 222 - DNA, 256 bp, synthetic construct
  source 1..256: mol_type = other DNA; note = iCDUPRT3-1-90 gene
acaaggacggcagtgtgctgggcagaggccacaatatgaggtttcagaagggcagtgccaccctgcatggggagatcagcaccctggagaactgtggcaggctggagggcaaggtctacaaggacaccactctgtacaccaccctcagcccttgtgacatgtgcacaggggccatcatcatgtatggcattcccaggtgtgtggtgggagaaaatgtcaatttcaagtctaaaggagaaaagtacctgcagaccag

SEQ ID NO: 223 - DNA, 399 bp, synthetic construct
  source 1..399: mol_type = other DNA; note = iCDUPRT3-2-98 gene
acatgtgcacaggggccatcatcatgtatgggattcccaggtgtgtggtgggagagaatgtcaacttcaagtcaaaaggagagaagtacctccagaccaggggccatgaggtggttgtggtggatgatgagaggtgcaagaagattatgaagcagttcattgatgagagaccccaggactggtttgaggacattggggaggcctctgagcccttcaagaatgtgtacctcctcccccagaccaaccaactcctgggactctacaccatcatcaggaacaagaacaccaccaggccagacttcatcttctacagtgacaggatcatcaggctcctggtggaggagggcctcaaccacctccctgtccagaagcagattgtggagactgacaccaatgaga

SEQ ID NO: 224 - DNA, 399 bp, synthetic construct
  source 1..399: mol_type = other DNA; note = iCDUPRT3-2-94 gene
acatgtgcacaggcgccatcatcatgtacggcattcccaggtgcgtggtgggagagaatgtcaacttcaagtcaaaaggagagaagtacctccagaccaggggccatgaggtggttgtggtggatgatgagaggtgcaagaagattatgaagcagttcattgatgagagaccccaggactggtttgaggacattggggaggcctctgagcccttcaagaatgtgtacctcctcccccagaccaaccaactcctgggactctacaccatcatcaggaacaagaacaccaccaggccagacttcatcttctacagtgacaggatcatcaggctcctggtggaggagggcctcaaccatctccctgtgcagaaacagattgtggagacagacaccaatgaga

SEQ ID NO: 225 - DNA, 399 bp, synthetic construct
  source 1..399: mol_type = other DNA; note = iCDUPRT3-2-90 gene
acatgtgcactggggccattatcatgtacggcattcctaggtgtgtcgtgggagagaatgtcaacttcaagtcaaaaggagagaagtacctccagaccaggggccatgaggtggttgtggtggatgatgagaggtgcaagaagattatgaagcagttcattgatgagagaccccaggactggtttgaggacattggggaggcctctgagcccttcaagaatgtgtacctcctcccccagaccaaccaactcctgggactctacaccatcatcaggaacaagaacaccaccaggccagacttcatcttctacagtgacaggatcatcaggctcctggtggaggagggcctcaaccatctccctgtccagaagcaaattgtggaaactgacacgaatgaga

SEQ ID NO: 226 - DNA, 394 bp, synthetic construct
  source 1..394: mol_type = other DNA; note = iCDUPRT3-3-98 gene
ttcatcttctacagtgacaggatcatcaggctgctggtggaggagggcctcaaccacctccctgtgcagaagcagattgtggagactgacaccaatgagaactttgagggagtgtctttcatgggcaagatttgtggggtgtccattgtgagggctggggagagcatggagcagggcctgagggactgttgcaggagtgtgaggattggcaagatcctgatccagagggatgaggagactgccctgcccaagctgttctatgagaagctccctgaagacatctctgagaggtatgtcttcctcctggaccccatgctggcaactggaggctctgcaatcatggccactgaggtgctcatcaagaggggtgtcaagcctgagaggatctacttcc

SEQ ID NO: 227 - DNA, 394 bp, synthetic construct
  source 1..394: mol_type = other DNA; note = iCDUPRT3-3-94 gene
ttcatcttctacagcgacaggatcatcagactcctggtggaggaaggcctcaaccacctccctgtgcagaagcagattgtggagactgacaccaatgagaactttgagggagtgtctttcatgggcaagatttgtggggtgtccattgtgagggctggggagagcatggagcagggcctgagggactgttgcaggagtgtgaggattggcaagatcctgatccagagggatgaggagactgccctgcccaagctgttctatgagaagctccctgaagacatctctgagaggtatgtcttcctcctggaccccatgctggcaactggaggctctgcaatcatggccactgaggtgctgatcaagaggggtgtcaagcctgaaaggatctacttcc

SEQ ID NO: 228 - DNA, 394 bp, synthetic construct
  source 1..394: mol_type = other DNA; note = iCDUPRT3-3-90 gene
ttcatcttctatagtgacagaatcatcagactcctggtcgaggaggggctcaaccacctccctgtgcagaagcagattgtggagactgacaccaatgagaactttgagggagtgtctttcatgggcaagatttgtggggtgtccattgtgagggctggggagagcatggagcagggcctgagggactgttgcaggagtgtgaggattggcaagatcctgatccagagggatgaggagactgccctgcccaagctgttctatgagaagctccctgaagacatctctgagaggtatgtcttcctcctggaccccatgctggcaactggaggctctgcaatcatggccactgaagtgctcattaagaggggtgtcaagccagagaggatttacttcc

SEQ ID NO: 229 - DNA, 477 bp, synthetic construct
  source 1..477: mol_type = other DNA; note = codon-optimized Fcy1 gene encoding cytosine deaminase
  CDS 1..477: protein_id = 230; translation = MVTGGMASKWDQKGMDIAYEEAALGYKEGGVPIGGCLINNKDGSVLGRGHNMRFQKGSATLHGEISTLENCGRLEGKVYKDTTLYTTLSPCDMCTGAIIMYGIPRCVVGENVNFKSKGEKYLQTRGHEVVVVDDERCKKIMKQFIDERPQDWFEDIGE
atggtcacaggaggcatggcttcaaagtgggaccagaagggcatggacattgcctatgaggaggctgctctgggctacaaggagggaggggtcccaattggtggctgcctcatcaacaacaaggatggcagtgtcctgggcaggggccacaacatgaggttccagaagggcagtgccaccctgcatggggagatcagcaccctggagaactgtggcaggctggagggcaaggtctacaaggacaccactctgtacaccaccctcagcccttgtgacatgtgcacaggggccatcatcatgtatggcattcccaggtgtgtggtgggagagaatgtcaacttcaagtcaaaaggagagaagtacctccagaccaggggccatgaggtggttgtggtggatgatgagaggtgcaagaagattatgaagcagttcattgatgagagaccccaggactggtttgaggacattggggagtga

SEQ ID NO: 230 - protein, 158 aa, synthetic construct
MVTGGMASKWDQKGMDIAYEEAALGYKEGGVPIGGCLINNKDGSVLGRGHNMRFQKGSATLHGEISTLENCGRLEGKVYKDTTLYTTLSPCDMCTGAIIMYGIPRCVVGENVNFKSKGEKYLQTRGHEVVVVDDERCKKIMKQFIDERPQDWFEDIGE

SEQ ID NO: 231 - DNA, 651 bp, synthetic construct
  source 1..651: mol_type = other DNA; note = codon-optimized Fur1 gene encoding uracil phosphoribosyltransferase
  CDS 1..651: protein_id = 232; translation = MSSEPFKNVYLLPQTNQLLGLYTIIRNKNTTRPDFIFYSDRIIRLLVEEGLNHLPVQKQIVETDTNENFEGVSFMGKICGVSIVRAGESMEQGLRDCCRSVRIGKILIQRDEETALPKLFYEKLPEDISERYVFLLDPMLATGGSAIMATEVLIKRGVKPERIYFLNLICSKEGIEKYHAAFPEVRIVTGALDRGLDENKYLVPGLGDFGDRYYCV
atgtcctctgagcccttcaagaatgtgtacctcctcccccagaccaaccaactcctgggactctacaccatcatcaggaacaagaacaccaccaggccagacttcatcttctacagtgacaggatcatcaggctcctggtggaggagggcctcaaccacctccctgtgcagaagcagattgtggagactgacaccaatgagaactttgagggagtgtctttcatgggcaagatttgtggggtgtccattgtgagggctggggagagcatggagcagggcctgagggactgttgcaggagtgtgaggattggcaagatcctgatccagagggatgaggagactgccctgcccaagctgttctatgagaagctccctgaagacatctctgagaggtatgtcttcctcctggaccccatgctggcaactggaggctctgcaatcatggccactgaggtgctcatcaagaggggagtcaagcctgagaggatctacttcctcaacctcatctgctcaaaggagggcattgagaagtaccatgctgccttccctgaagtgaggattgtcactggggctctggacaggggcctggatgagaacaagtacctggtccctggcctgggagactttggggacagatactactgtgtctaa

SEQ ID NO: 232 - protein, 216 aa, synthetic construct
MSSEPFKNVYLLPQTNQLLGLYTIIRNKNTTRPDFIFYSDRIIRLLVEEGLNHLPVQKQIVETDTNENFEGVSFMGKICGVSIVRAGESMEQGLRDCCRSVRIGKILIQRDEETALPKLFYEKLPEDISERYVFLLDPMLATGGSAIMATEVLIKRGVKPERIYFLNLICSKEGIEKYHAAFPEVRIVTGALDRGLDENKYLVPGLGDFGDRYYCV

SEQ ID NO: 233 - RNA, 477 nt, Saccharomyces cerevisiae
  source 1..477: mol_type = mRNA
atggtgacagggggaatggcaagcaagtgggatcagaagggtatggacattgcctatgaggaggcggccttaggttacaaagagggtggtgttcctattggcggatgtcttatcaataacaaagacggaagtgttctcggtcgtggtcacaacatgagatttcaaaagggatccgccacactacatggtgagatctccactttggaaaactgtgggagattagagggcaaagtgtacaaagataccactttgtatacgacgctgtctccatgcgacatgtgtacaggtgccatcatcatgtatggtattccacgctgtgttgtcggtgagaacgttaatttcaaaagtaagggcgagaaatatttacaaactagaggtcacgaggttgttgttgttgacgatgagaggtgtaaaaagatcatgaaacaatttatcgatgaaagacctcaggattggtttgaagatattggtgagtag

SEQ ID NO: 234 - RNA, 651 nt, Saccharomyces cerevisiae
  source 1..651: mol_type = mRNA
atgtcttcggaaccatttaagaacgtctacttgctacctcaaacaaaccaattgctgggtttgtacaccatcatcagaaataagaatacaactagacctgatttcattttctactccgatagaatcatcagattgttggttgaagaaggtttgaaccatctacctgtgcaaaagcaaattgtggaaactgacaccaacgaaaacttcgaaggtgtctcattcatgggtaaaatctgtggtgtttccattgtcagagctggtgaatcgatggagcaaggattaagagactgttgtaggtctgtgcgtatcggtaaaattttaattcaaagggacgaggagactgctttaccaaagttattctacgaaaaattaccagaggatatatctgaaaggtatgtcttcctattagacccaatgctggccaccggtggtagtgctatcatggctacagaagtcttgattaagagaggtgttaagccagagagaatttacttcttaaacctaatctgtagtaaggaagggattgaaaaataccatgccgccttcccagaggtcagaattgttactggtgccctcgacagaggtctagatgaaaacaagtatctagttccagggttgggtgactttggtgacagatactactgtgtttaa